European Patent Application EP 4 632 067 A1, published October 15, 2025. Title: METHOD FOR PRODUCING GENOME-EDITED CELLS AND METHOD FOR PROMOTING HYBRIDIZATION. Applicant: TOKYO UNIVERSITY OF SCIENCE FOUNDATION. The sequence listing filed with the application follows.

SEQUENCE LISTING (91 sequences)

SEQ ID NO: 1 - DNA, 748 bp, synthetic construct
  source 1..748: mol_type = other DNA
tgtggaccagacaggcgccactcggccgggccacaactgcttgggttttgaccgggagcggaccaattaaggactcgaacgaccgcggggttcaaatgcaaacaagtacaacacgcagcaaacgaagcagcccaccactgcgttgatgcccagtttgtctgtccgaaatccaccggaaaggtggaaacatactatgtaacaatcagagggaagaaaaattttttatcgacgaggcaggatagtgactgatggtggggtcatggtcgggtctccgagcgaaagagaaccaaggaaacaagatcaacgaggttggtgtacccaaaaggccgcagcaacaagagtcatcgcccaaaagtcaacagtctggaagagactccgccgtgcagattctgcgtcggtcccgcacatgcgtggtgggggcattacccctccatgtccaatgataagggcggcggtcgagggcttaagcccgcccactaattcgccttctcgcttgcccctccatataaggattcccctccttcccctcccacaacttttttcctctttctctcttcgtccgcatcagtacgtatatctttcccccctacctctttctcactcttcctcgattcattccactcttctccttactgacatctgttttgctcagtacctctacgcgatcagccgtagtatctgagcaagcttttttacagaatctttctagtatcttacaaagaactacaaagttcgcaccaccttcaaa

SEQ ID NO: 2 - DNA, 1168 bp, Aspergillus sojae
  source 1..1168: mol_type = genomic DNA
atggaaaccacagtgtctcccctccagcgtgcgtttaacgcattcttgatgaccatgccacccgagcagttggaggagctgctcaagtacctccaggacgcaaaatctcaggaaaatactcaatcttcatatccgaaagaaaatcttcaatcttgcttggagttcaaggcagacaaaaacaatggatctaccaaccctgcgagtgctaacccacggtcctcagcttcgcgggggaagcgtgcctcagatgcaaaacgaaggccgctcaatagtttcattgcctttaggagtgagtgtccttgtaccgtgatcgagcgaattccacattctaacaatactaggctattactccatcatgttccctgacctcactcagaaggcaaagtcgggcattcttcgcttcctgtggcagaacgatccattcaaagccaaatgggcaatccttgccaaagcctactccatcgttcgcgatgaccacgatagtgatgtttctctggaatcttttttgggtttgaatgcacagttcattggtataattggaccaagtcgttatcttgaagttatgggctggcaactggatgtcgacgatcagcaacaatatactatagctagggttaaagcgacgactgcaaatgaagccgatatttcgaccaactattctgtcaatgatatagttaaacattgctacaccagtggctatgtttccgagaaaaatcggaagagcaaggcaagcaataacaacagtgccccggttatggcttttgctgcccagccgaccttggttgtccacaagaacgacagtattcgggtatctggcaaccatactattgtaaccgatgtttacaaaacgaatccagctatggaaatatcttcaccggagcaaactgaagatacattttcgccaaacactagtgacttgagcacaattgctgatgaacctccgctcgatgcaatggaagtagtgggtatctgcaaccgccctcagctttactcggattcaagtacgccgaattgttttgatttcgataacatccaattcccaggctgggatgaggagaacgcaatgttcacttacgatgccgcactacaaacgccactgatgccctatgatccgctgaactacgatccactggaagcctatgacttctctagattcgttgatatttga

SEQ ID NO: 3 - DNA, 1069 bp, Aspergillus oryzae
  source 1..1069: mol_type = genomic DNA
atgacgactatacctatcgctatgaagacgaccgcggagtcgacggacaagcttacagagctgctttggcaggatgctttgcgtcacctcgagtctacaaataatgaggtgcttttgccgattaatgtcacagacatgataggtcaaagcaatgtcgacaagattaggactcgtctcgggtaagaagagttctcagattctctaggtatacaaacttacatttggtgatagtgctcttatcggtgctcctgtggtggcttttgtcgatgagacgatcaatgctctccgtgtaatgcgcacgcctgctttttcgggctccgttgtgtccgtcgcatctcatgacagaatttcgaacttagaaaaggaaatcaccgaagcatctggtagaacacatggcaaatccgcactaccaacgaagtccaaagtccctcgaccaccaaatgcattcatcctttatcgtcagcatcaccatcccagaatcaaagaagcatatcccgatttcaccaataatgagatatgtaagtttccttttcatctctactcaacttcgaacaagctaacgacatcagcaatcatccttggaaaacaatggaaggccgaatccgaagaggtcaaaatgcaatttcgcaatatggcggagaaacttaagaaaaagcatgcagaagaccaccccgattaccattatactccccgcaagccatccgaaaagaagcgtcgagcttcgtcccgccagtactctaagccgaccaaacgacagaagtccccggccttgacaaatgatacctctgatagctccacaccgtcgatgtactccggcatgcagctggacaacatacctgtagatgcatctttggataatttggctgatatcgacatcgtgctcagccccgatgaactgcctagggactgtgggctacaattcgactcagttgccttcgataattttctccagcaagtacagggcgactgtggcaagacagccgctactttgttcccacagttcaacttcacagaaaggcctgtgggagagtcattcgaattttcagatttgattgctgactgctactga

SEQ ID NO: 4 - DNA, 800 bp, synthetic construct
  source 1..800: mol_type = other DNA
gtaccaggagtacattggagagttctaccattgttgctggaatacaatgatgattagaaaccgaagagtgttatgattcggacggatatacgcatggcacgcatacagcgtgatacataggctgtttgctcaagaattaggattttatctgaatccatgtacagagtttacttatgttagtagtcaatgaaatcttggctttctaattttgtccgatctacaaggggtagtcgatcacagaacgaactagatgtgcagggaacgatgatcacccgctcttagcaagacctctagtagttttcgaccatagctttaacgcgaatcatgaccctactattttctagattgcagaccaagtcacatgacaatgtcctctttgaagtaggatcagtagctgattagattccgggaaatgaattagggctggcgttccaactactggggagtgccgatgttgctgtatgaaagatagtaagattactagtgcacagctgtagtaattatttactctagattatatattccaaataataagtaatctaagatagtagacagtcctatgatatagctccgggttcgaagtcggcaaaagatatgcaatcacctgtcgggatgatatatgtatatctgaaataccgacatcaaccatccagtcggatcagctaaacgaagtatcacttctttcgccactgccaatcactacttctattaaagttcatgttacagtataagccacaagacttatctccagaactaacttgtgcataggagctctgccgatagccgggtggttggatcgg

SEQ ID NO: 5 - DNA, 37 bp, synthetic construct
  source 1..37: mol_type = other DNA
cggtacccggggatctgtggaccagacaggcgccact

SEQ ID NO: 6 - DNA, 25 bp, synthetic construct
  source 1..25: mol_type = other DNA
tttgaaggtggtgcgaactttgtag

SEQ ID NO: 7 - DNA, 40 bp, synthetic construct
  source 1..40: mol_type = other DNA
cgcaccaccttcaaaatggaaaccacagtgtctcccctcc

SEQ ID NO: 8 - DNA, 42 bp, synthetic construct
  source 1..42: mol_type = other DNA
atgtactcctggtactcaaatatcaacgaatctagagaagtc

SEQ ID NO: 9 - DNA, 25 bp, synthetic construct
  source 1..25: mol_type = other DNA
gtaccaggagtacattggagagttc

SEQ ID NO: 10 - DNA, 39 bp, synthetic construct
  source 1..39: mol_type = other DNA
cgactctagaggatcccgatccaaccacccggctatcgg

SEQ ID NO: 11 - DNA, 40 bp, synthetic construct
  source 1..40: mol_type = other DNA
cgcaccaccttcaaaatgacgactatacctatcgctatga

SEQ ID NO: 12 - DNA, 40 bp, synthetic construct
  source 1..40: mol_type = other DNA
atgtactcctggtactcagtagcagtcagcaatcaaatct

SEQ ID NO: 13 - DNA, 1009 bp, synthetic construct
  source 1..1009: mol_type = other DNA
agcaaacggtggtcaaaggatggttcagatacaaattagcaacaggccaggctagacgcgcgactatccactgcggcaaatggtgagctgcaagcaacggtaagatgtgacaggacgagcggtgtgccgggaaaaaaattggaggagcgcaaagcggcggctgtccctcagtggtgcccaaacgttatcgatagtacaccaagcatgggcagtgagcggctatacagagggaataataggcatatcggcacgactagattcggtagaaagcatcgaagagcaattcattgagcatattatcacgtggaatgcgatagctgtggccaggttgagacaccgcaagtgaaagatacacacatagattctcgattcgagcggtttgcctccgccaccgcagtgcatagcaagcaaagaaacgacagttggctcatcatccgttacatcattttttctactggctccgctcggtgggctcccaacgaagcagcaaaaaagtgagagaaaaaaactagcttggcggggcaacagaagctagaccctttggctcgcttagtcagtgcgcccactcactcacactcaaaaaggccacccctcccgcaccctcttctcatcaccgtcttcataccacggttcgtcaagcaatcgtatctggtaagctttgacctcctcgagcgggctccactttgctatttcttggatctgctctttcttttctctctacctctttttctaacctctcttcagaaagttcaaccgtacttcactcaatcttccatacacaaccgtcggcgcgccgctagcttaattaaacaatcaatccatttcgctatagttaaaggatggggatgagggcaattggttatatgatcatgtatgtagtgggtgtgcataatagtagtgaaatggaagccaagtcatgtgattgtaatcgaccgacggaattgaggatatccggaaatacagacaccgtgaaaggcatggtctttccttcgtgtagaagaccagacag

SEQ ID NO: 14 - DNA, 30 bp, synthetic construct
  source 1..30: mol_type = other DNA
attgtatctgaggaaaggaagaggggaaac

SEQ ID NO: 15 - DNA, 35 bp, synthetic construct
  source 1..35: mol_type = other DNA
ttttaacagaggaaaaacccaatgattcagtcttt

SEQ ID NO: 16 - DNA, 30 bp, synthetic construct
  source 1..30: mol_type = other DNA
ccagcgaagaggacgaagacaccacatgga

SEQ ID NO: 17 - DNA, 35 bp, synthetic construct
  source 1..35: mol_type = other DNA
atgaagccgttgacacacttcttcttcatctgggg

SEQ ID NO: 18 - DNA, 20 bp, synthetic construct
  source 1..20: mol_type = other DNA
cagccttccttcctgggcat

SEQ ID NO: 19 - DNA, 20 bp, synthetic construct
  source 1..20: mol_type = other DNA
cattgtgctgggtgccaggg

SEQ ID NO: 20 - DNA, 1504 bp, Pyricularia oryzae
  source 1..1504: mol_type = genomic DNA
atggattcattgcagatggactcctctcaaatggaggcgttgtcgtcgatttgggtcatcgtgcagcatcagctcgcccaaatcaacaattccaacaacatagctcatatcggcgccgttctcctcaaccaacttgaggcgcctttcaggagcactttgacatcatggtttcagcagtaagttctccataagctcaaggcttttccgcaagggaaactaacatcaggtaggcacaccggcatcaaccaggtctcagtcgtgcgcgacatcaaggctcgtcgacactacatcggaccaactgatgcttttcaggagagctatcaagttgtacacatccagggtcacggatttgtctggctttgggatctccaggttgatggtgaggatgccagcatcaattcctgcaatatctctgccgagacagcacagaacttttcccagctgcgtcttgacgagatggcgcctaccaatgatgttacgatggtaggtgatgagagcctcatcaacggcaacggcattgactttgccatgttggaagacatcggaagccccgcatcaaacggctcctcattcccgagccctcaagttttcacccgggaaatttcattcgatgatctaccagttggcattatgactgccgaggccattcagagagaccttcttggcgccaatattcgcccggctaacctcattgatccgagtcttgcgagcaatcagaatgtccacaacatcatccatcagaataacattgcccaggcttttacagatcacctgaacatgatggcatccaatgctgtccacgatgacacagaagagggtctgacagccgcggatcttatgccggcgttgcatcgcatgttcgtgccgggtcttgagtcaattgcaatggagcagttccacaccacgcttcctaatggcgcactccttcacctgtcaattcctgtcgatgaacctgaggatgctgtctcgaccaccgcgcctgctgctcaacagacttccttgcaagacaagatccctcgtcctgcgaatgcctacatcctgtaccgcaaggattggcatcccatagtcaagtctgcaaatccaggaatccataacaacgaaatctgtgagttcttttacctccaaacttccctagctgctgctaactttttttcctttagcaaaaatcctggggaagcagtgggcagctgagacaccggaagtgcgggctgagtacaaggagctcgcggaggagaagaagagagagttctacgcaaagtaccctacatatcgctactctcctcgtcggccgagtgagataatgcgccgagtgagtttgtaacacattattgcgtgaaagagtggacagcgagctaacaaattacttgccaacaagaacacgaaaagccgaaagaccccaacgaacggggcagcgaagccgagcaaagcaaagaagtgcggcaacggggttactggtggagcagacagtgcagtcgatgtcagctccccgggatcgccattttag

SEQ ID NO: 21 - DNA, 40 bp, synthetic construct
  source 1..40: mol_type = other DNA
gtgaatggtttaattaactaaaatggcgatcccggggagc

SEQ ID NO: 22 - DNA, 35 bp, synthetic construct
  source 1..35: mol_type = other DNA
cgaggcaggcgcgccatggattcattgcagatgga

SEQ ID NO: 23 - DNA, 1171 bp, Pyricularia oryzae
  source 1..1171: mol_type = genomic DNA
atgccggccctctggtcaccagtcaaagtttgcggcatcgtttcggagctcaggtaagccgacccagagtcctcacaccagagcgacagctcttcagcatctaacgatcacaggctaacacttttggcgcctcaattagcaagaacatggcctgcatggtttggatctgggtcgtctgcgttcctcagaagcggtaccgcatcacgacagctcgctggaactccagtgggctgctggttggccgcgttgattgtgagttttctactttcttcaccttttccttccgtcccagatctgagcagagactgacaagcgacacaaaacctccccacagctcctcctcaatctgccaccacagcgtcctcacagtcatcgtcattcgacggcagtgaggaagacacaaacacaaacatcaacgccaatggtatcgatgagagcctgctgccgcctgctctccgcggccgcactggaccttccaagcctccaaaccgctggattctctaccgtgccgccaagtcagctgagctgcgggcagacaacccatccatgaacgcgagcgaaatctgtaagttcttcgctcttttcactctttttctccgctaccacttgtacctaccttttccccatctcccatactctttgaaaagtctccagtcccacctctcaagctgctgttttgacaagataaaagactaaccaacatctctctcctcacacagctcaagttgcatccctgatgtggcaggcagagtccgccgcgacaaaggcagagtgggaggagcgcgcagccgaagcccgcgaggagcacatgcgaaacactccagagtatgcggtggcggccggtctgcgccagcgcgccatcgccgagaggagaaggcagaggcagcagaagaagaagcaacaggagcagcagaagggcgacggtgacaaggtggccaaggagacttctacatccacagagagcttggtcactacggacgtcggcgctgtcagcaaccacggcagcagcagcagtgaggtgcctgtcacaagcccacactcgccgacactactcagtcccgcgtctgacagcgattgtacgcccgtcggcagccctcgagctcgccacggctggggttctgatgctctcagcctgatgctcgacgccgccgaattctctactctcttctga

SEQ ID NO: 24 - DNA, 34 bp, synthetic construct
  source 1..34: mol_type = other DNA
cgaaagaaggcgcgccatgccggccctctggtca

SEQ ID NO: 25 - DNA, 47 bp, synthetic construct
  source 1..47: mol_type = other DNA
cagagtgccagttaattaatcagaagagagtagagaattcggcggcg

SEQ ID NO: 26 - DNA, 1037 bp, Pyricularia oryzae
  source 1..1037: mol_type = genomic DNA
atgattgccagtctctcgcctgacgacatcgccaggctgattccccaggagactctgacttctctgctcagagcaaatgacgagaaagagcgcctgcgggagctgcccgttagcccgagagcggtagcagcggcgagcaaaaacaagaagaaagtcaatggatttatggcatttcgatgtgagtacagactgataatagagaaatcgaagcttgtgctgacagcagtatagcctactacgctggcatctttcaggatagaccgcagaaagaacgttcgcccttcatcactctactctggcagaaggaaacgctcaagtcaagatggactctcatggccaatgttttctctcgcattagggactttgcaggcaccacaagaggtcgtatggcaatgagtggattcctgcgagttgcctgcccgcttctgggcatcaccaaaccctgcgactacctcagacgctacaattgggaactcgagtttgttgcagacgcgtcagctccgtatgatgctgctatgaaatacgagatttcccagtcacaaatccctcacattgtcgacgaattcgaggtccctactacggagattgagttgcttcgcgcctgcgttcagggtggctttccatttgagaacagtgcccagcttctaagagacatggaagacagctctgtcaccgttatgaccagaactgcgcctatcatggcaccctcgcatgcttcgcaggcctcgcatggccaacataaccaccatttcatcaacacactcatcaacgacccggatgctgcgatatctgcgcttttgccccaagatgaagacattggcagtctgatggttgacatgaatatcatccactcactcgagacagacagctcaacaacatcatcggcacgcaactcagtttctcctctggagcagcacttgttctttcacgaagacgtctccatcgatccttcaacaatggtttctttccctggcgaaggtcatggtcacccggaaacacaatacagctaccccaatccaacgctaggtctctggtaa

SEQ ID NO: 27 - DNA, 34 bp, synthetic construct; identical to SEQ ID NO: 24
  source 1..34: mol_type = other DNA

SEQ ID NO: 28 - DNA, 44 bp, synthetic construct
  source 1..44: mol_type = other DNA
cctgagatttaattaattaccagagacctagcgttggattgggg

SEQ ID NO: 29 - DNA, 966 bp, Pyricularia oryzae
  source 1..966: mol_type = genomic DNA
atgtcaactgcatcagattatctatacataaagattcctcccttcaacttctacaagaatggaaaaccagagccagaggatattgctgtctatcgagcgcgcccgtttgtatctgcatgcaagacccttctcggttctgtcgcggaactcttaggcgatagcagcatgaaccaaaacaccgagtgccatcaagccattgtctctgctttgcaagcaaccaaagagttttttaccctgcaagcattattagacacactgaaggcttacaaagacggctctgagcctcttccaaagaagtggacagagcagagcctgcagggtgctttacaccgagcccgatgcgccatacgtgattcagatcacgcccgaaagctcagctatgctatttcgctttgcttcgatttatctcagcgaaccaaggttaactcaggcaatacctgtcttctggccgccgtggtgacccttctggcaatgagggtgcggacactccagtatgagccagttgctcagtctgtcagcgcttctattggccttctcagggtccaagatggttgccttgttctcagagagcacagtcatcctaaggactacgggcaatggcttgatattatcgagcacccctctcttccaacaatgccgggcagccgatggggcctgtttcatcgggtcctagacctgcctttcttcgatcaagaaaagctgcgcgattttactttcataacaactcactgcgccaactccttgatacgttctacaatggggtgctacactaccgcacgtcagcaagctgctacactgcgtgaaagcgtcatacgcttgagctatgaagatgagcaggtatgcactctaacatgtccctgtatttacactgctaactttgagaagaccaagataaagattgcaaatgatcgcgcgcggctacctctaaatcctccagtggtaggcttgttgactcttctattttga

SEQ ID NO: 30 - DNA, 35 bp, synthetic construct
  source 1..35: mol_type = other DNA
cgtcaggcgcgccatgtcaactgcatcagattatc

SEQ ID NO: 31 - DNA, 40 bp, synthetic construct
  source 1..40: mol_type = other DNA
gtaatgttttaattaatcaaaatagaagagtcaacaagcc

SEQ ID NO: 32 - DNA, 1265 bp, Pyricularia oryzae
  source 1..1265: mol_type = genomic DNA
atggactacgagaacagcatagtggcgagccagatgcctgcagagaggatatctgtcagcgtctcgatacctcaacaaacagttgatttcgaggtgccggccctctggtcgctaggcaaagtttgcggcatcgcttcggagctcaggtaagccgacccagagtcctcacaccagagcgacagctcttcagcatctagcgatcacaggctaacacttttggcgcctcaaattagcaagaacatggcctgcatggtttggatctgggtcgtctgcgttcctcagaagcggtaccgcatcacgacagctcgctggaactccagtgggctgctggttggccgcgttgatcgtgagttttctactttcttcaccttttccttccctcccagatctgagcagagactgacaagcgacacaaaacctccccacagctcctcctcaatctgccaccacagcgtcctcacagtcatcgtcattcgacggcagtgaggaagacacaaacacaaacatcaacgccaatggtatcgatgagaacctgctgccgcctgctctccgcggccgcactggaccttccaagcctccaaaccgctggattctctaccgtgccgccaagtcagctgagctgcgggcagacaacccatccatgaacgcgagcgaaatctgtaagttcttcgctcttttcactctttttctccgctaccacttgtacctaccttttccccatctcccatactctttgaaaagtctccagtcccacctctcaagctgctgttttgacaagataaaagactaaccaacatctctctcctcacacagctcaagttgcatccctgatgtggcaggcagagtccgccgcgacaaaggcagagtgggaggagcgcgcagccgaagcccgcgaggagcacatgcgaaacactccagagtatgcggtggcggccggtctgcgccagcgcgccatcgccgagaggagaaggcagaggcagcagaagaagaagcaacaggagcagcagaagggcgacggtgacaaggtggccaaggagacttctacatccacagagagcttggtcactacggacgtcggcgctgtcagcaaccacggcagcagcagcagtgaggtgcctgtcacaagcccacactcgccgacactactcagtcccgcgtctgacagcgattgtacgcccgtcggcagccctcgagctcgccacggctggggttctgatgctctcagcctgatgctcgacgccgccgaattctctactctcttctga

SEQ ID NO: 33 - DNA, 36 bp, synthetic construct
  source 1..36: mol_type = other DNA
tcatcgtggcgcgccatggactacgagaacagcata

SEQ ID NO: 34 - DNA, 41 bp, synthetic construct
  source 1..41: mol_type = other DNA
gtgccagttaattaatcagaagagagtagagaattcggcgg

SEQ ID NO: 35 - DNA, 1199 bp, Pyricularia oryzae
  source 1..1199: mol_type = genomic DNA
atgacgcaggttgaggatgactacgatgagagcgccaatgcggatgagagcggcggggctggtccaggagcacctacgcctctgactgctttggaggtatgctttgcccgataaactccgtagaagtcgtcctcgctaatgtattgatgaaatcattcagggcgttggaggcctaacaaagagggatattcaactggtcatggaaggtggatacaacaccgtagagtctgtcgcctacacacccaggcggatgttggagcaaatcaaaggaatctcggaacaaaaggcaggaaagattctcgcagaaggtaagatgagttgatgtgatacaaccagaatgacctgcctcaagcctcgtcactaaccacaccctgtcaatagcatccaaacttgtacctatgggcttcacaacggcgactgagatgcaccagcgcagaagtgagctgatatcgatcacgactggttcgaagaacctcgataccatgctgggtggaggtatcgagaccggctctgtcacggagctctttggagagttccgtacaggaaaatcacagatttgccacacgcttgccgtgacatgccagttgccctttgatatgggcggcggagagggcaaatgtctatacatcgacaccgagggcacattccggcccgttcgactgctcgccgtggccaaccgctttggattgtcgggcgaggaggtgctcgacaacgttgcctacgcacgcgcgtacaactccgaccatcagcttcagcttctgaaccaggcttcggccatgatgtgcgaaacgcgcttcagtctccttattgtggattctgccaccgcactgtaccgtaccgacttccttggtcgtggagagctgagcagtcggcagactcatctagcaaagttcatgcggcagctgcagaggctggcggatgagtttggtattgcagttgtcatctcaaatcaggttgttgcacaggtcgatggtggtccctcggccatgttcaaccctgatcccaagaaacccataggcggtaacatcatcgctcacgccagcactaccagactgagtctgaagaagggtcgcggcgagaccagaatcgccaaaatttatgacagtccatgtctaccagagagtgactgtctattcgccatcaatgaggacggcattggtgacccttcgccgaaggatgtcgagaagatgaacaactga

SEQ ID NO: 36 - DNA, 35 bp, synthetic construct
  source 1..35: mol_type = other DNA
aaaggcgcgccatgacgcaggttgaggatgactac

SEQ ID NO: 37 - DNA, 35 bp, synthetic construct
  source 1..35: mol_type = other DNA
aaattaattaatcagttgttcatcttctcgacatc

SEQ ID NO: 38 - DNA, 1353 bp, Pyricularia oryzae
  source 1..1353: mol_type = genomic DNA
atggcttctttacgaggcatgtgggctccagcagccgtacgtgtccttcgtcaggccgtcggcagtactgtcaaaatatcgaaagtgctgcgcaccaagctgggaagcgcagcacaccgaccgatcacccagcttcctcagcctgttacatctgcagctaggcaccaacccatccacccattcgcatttctgcgccagcagaaacgcggtttccgatggcactccgcccttcgcaacactcactatgatgccgtacgaaacacccttcgtcgcttcatcagtgggtcagcacgtgcccagccttcgcagtcgggccagacaacacgctgggttaagcagttcacaggtcgtgctccttttgcgtcgacgctgcgtccgaacttgaccggaggtgcattcccgagaaccgccggcgggtatgcgatgccaggatctggaaagatgggtggtgcacgctatttcagccatgcaccccctgtgcaagctcaggttatgcaaaatgttgggcaggcaatgcgggctttctggctctcgggccagcgcgcgcactttgacggatatgggcctcggggagagaagtgctatcgtgtcaccaccgagttgcaggacgagaccgcgaggaaggccgcatcagctgctgcatcacacaagcgtgtgccgggttccttcattgacttttctgtcaatcctaccatcacggcactcagcccccttgccggtaacttccccttcgctatgcgcggtatcgaacaagaaaccgcagtcaatggccccacgttgaaccaagatgggctcctcgatctgctcttgaccgatttccagcgtgcgttcaaggatcttaatgctgtcatggcagatctaaagaggctctcaaatcttggagatctaccaatcgtcttcgagaatgattctcaccttgtacgtgttcggttcccaggtgtggatgcggatactgtaacgaggctctgcgaagatattggcatccaacaggggattgttggacaggacgaagacttcaagacggcccaggactatccatcggacctgcgcttcccatttgcgcctgaccacggcaatccaaaccacttatcttcgcctggtgggtctttgagatctcatcaatcctactcatcagatctgtcaattgatttggatgatgagtatgtggagcattttatggaggagaacccttggctctcctcagtagatgcagatgaatataaccattctcgcatcagcctagtctcacccactccggacaggcaaatcaactcacagttacaggacttcgagggcgtggaaggcatttatcgatttatacaagagtgtgatcgagctgctgggcgtctttga

SEQ ID NO: 39 - DNA, 35 bp, synthetic construct
  source 1..35: mol_type = other DNA
gtcggcgcgccatgacatccccaaacaacccccca

SEQ ID NO: 40 - DNA, 35 bp, synthetic construct
  source 1..35: mol_type = other DNA
gtttaattaactacggcccgggggcagggcgagta

SEQ ID NO: 41 - DNA, 588 bp, Pyricularia oryzae
  source 1..588: mol_type = genomic DNA
atgacatccccaaacaaccccccagaccacaaagccctcatggcccaagccctgaccctcgccagatcctcgccgtgcctacccacaaactaccgcgtcggcgctttgctagtcgacccatccccttccacagcatcatcacaagaaccctccaccccctcctcccccacagtcctcgcaacaggctacaccctcgagctcccaggcaacacccacgcggagcagtgctgcatcgccaaggtctcctcgccagcagccgacgcaccacccagcaccgagctcccaggcgaccagcaaatacagcaactagccctgcccaggggccggctggccctgtacacgaccatggagccgtgcgtggagcgcctgagcggcaacctgccgtgcgtgcagcgcatcctcgcctaccgggactttatcaccgacgtttatgtgggcgtgctcgagcccgacacctttgtcaagggcaactcgggccgcgccgtgctagaggccgctggtgtcaaggtgcatcacgtcgttggtctcgaggatgagattctcgaggttgcaaccgccggccatactcgccctgcccccgggccgtag

SEQ ID NO: 42 - DNA, 35 bp, synthetic construct; identical to SEQ ID NO: 39
  source 1..35: mol_type = other DNA

SEQ ID NO: 43 - DNA, 35 bp, synthetic construct; identical to SEQ ID NO: 40
  source 1..35: mol_type = other DNA

SEQ ID NO: 44 - DNA, 733 bp, Pyricularia oryzae
  source 1..733: mol_type = genomic DNA
atgtcgctcccgccctcgatccaaaagctgagcagcagcgacgacgcggcggtggatgaagtctgcaagacgtacggcatcagcagggagcagttccagcagttgcaacgccgcagcgaggcggcaaagtcgacggcctactgcccctacagcaacttccgcgtcggcgccaccctgctttcaatcgacgacaagaactcgtacataagcggcgccaacgtcgagaacgcatcgtacccagtcggcacgtgtgccgagcgcgtggcccttggcaaggccgtcaccgagggtcaccggcgattcagggccctcgcggtgtccacagacatcactccgccggcgagcccgtgtggcatgtgcaggcaattgtcagtatttctttttgcttaccccccgcttgtgctccgcatccgatcggggattcaatcccggaccagtgatgggatctaggtggataccacacccccgtctggagccccggcgccctttccgggaatttgctgggagtatttgtttatgggaccccaccattgtccagaagatcggcttgctgtttttagttttttttttattgttacaaaactgacctcgccaccctcactccagcatccgggagttttccgacttgcatatgcctatattcatgttcgataaggacaatgactttgtggttatgaagcttgaggctgtaagataccccgccgccaccaacatcggcatgtttggtttttaa

SEQ ID NO: 45 - DNA, 33 bp, synthetic construct
  source 1..33: mol_type = other DNA
gtcggcgcgccatgtcgctcccgccctcgatcc

SEQ ID NO: 46 - DNA, 35 bp, synthetic construct
  source 1..35: mol_type = other DNA
tgtttaattaattaaaaaccaaacatgccgatgtt

SEQ ID NO: 47 - DNA, 1294 bp, Pyricularia oryzae
  source 1..1294: mol_type = genomic DNA
atgtccaccctcaagcgcaaggccaatggaccgctgtcagcttcagatgccaagaaacccaaacagaacgccagcatcacatcattctttgccgcacctaagaccacaccggccagcggcgccaccacatctagcagcccaagttctacagcggcgccagcagcctcagctccagcccatccaccggctgtcagtttcaacaagcagaaatgggtggagaagcttaccaacgagcagagggagctgctaaagctggagattgacactttggacgagagctggcttgcgttgctcaaggacgagattaccacaaaggagtttcttgacctgaaaaggttcctagacagggaagcgaatgcgggcaagaaggtgtttccaccaagagaagatgtctactcatggtatgtaaaccggcgagcctcgttaccgtcacaagcggacatatgcgtcactatgttctgttgtatagaggtattgacatgttccgtttcgttttgccacacacaggtcccgccatacgcccttccacacagtcaaggtcgtaatacttggccaagatccttaccacaatatcaatcaggcccatgggcttgccttctcagtgcgaccaccgactaaggcaccaccatctctcaaaaacatgtacatttgcctcaagaacgactaccctgaattcacgccgccgcccaacaactcgggcctgctaacgccctgggcccagcgcggcgtgctgatgctcaacacatgccttacggtccgggcgcatgaggccaattcgcacgcaaaccggggctgggagaagtttacgcaaaagatcatcgagctcgtggcgggtcgtcgcagcaggggcgttgtattcatggcttggggtagccccgcagctaagagggtgatcaaggtcgaccagaagaagcacttggtgctcaaagcggtgcacccgagcccattgagcgcgtcaaggggattctttgactgcggtcactttagaaaagccaacgagtggttggtgcagaggtatggggacggggaggagatcgactggagcctaacggagggagtcagcctcttgcccaagccaaaggtcgaggtggtcaaggcggcacccgaggcaaagaaagtcaagaaagatgaggaggagtttgactttgacgaaggggaagagcttgaggcgctggaggagttgcgaaagatcgaagacaacaagaagcccgaagttccagcacctttgactgcgaagccaggggtcgaggtcaaaggagacgagaataagaatccttctacggctacagcatga

SEQ ID NO: 48 - DNA, 35 bp, synthetic construct
  source 1..35: mol_type = other DNA
gtcggcgcgccatgtccaccctcaagcgcaaggcc

SEQ ID NO: 49 - DNA, 36 bp, synthetic construct
  source 1..36: mol_type = other DNA
tgtttaattaatcatgctgtagccgtagaaggattc

SEQ ID NO: 50 - DNA, 2042 bp, Pyricularia oryzae
  source 1..2042: mol_type = genomic DNA
atgtccaccctcaagcgcaaggccaatggaccgctgtcagcttcagatgccaagaaacccaaacagaacgccagcatcacatcattctttgccgcacctaagaccacaccggccagcggcgccaccacatctagcagcccaagttctacagcggcgccagcagcctcagctccagcccatccaccggctgtcagtttcaacaagcagaaatgggtggagaagcttaccaacgagcagagggagctgctaaagctggagattgacactttggacgagagctggcttgcgttgctcaaggacgagattaccacaaaggagtttcttgacctgaaaaggttcctagacagggaagcgaatgcgggcaagaaggtgtttccaccaagagaagatgtctactcatggtatgtaaaccggcgagcctcgttaccgtcacaagcggacatatgcgtcactatgttctgttgtatagaggtattgacatgttccgtttcgttttgccacacacaggtcccgccatacgcccttccacacagtcaaggtcgtaatacttggccaagatccttaccacaatatcaatcaggcccatgggcttgccttctcagtgcgaccaccgactaaggcaccaccatctctcaaaaacatgtacatttgcctcaagaacgactaccctgaattcacgccgccgcccaacaactcgggcctgctaacgccctgggcccagcgcggcgtgctgatgctcaacacatgccttacggtccgggcgcatgaggccaattcgcacgcaaaccggggctgggagaagtttacgcaaaagatcatcgagctcgtggcgggtcgtcgcagcaggggcgttgtattcatggcttggggtagccccgcagctaagagggtgatcaaggtcgaccagaagaagcacttggtgctcaaagcggtgcacccgagcccattgagcgcgtcaaggggattctttgactgcggtcactttagaaaagccaacgagtggttggtgcagaggtatggggacggggaggagatcgactggagcctaacggagggagtcagcctcttgcccaagccaaaggtcgaggtggtcaaggcggcacccgaggcaaagaaagtcaagaaagatgaggaggagtttgactttgacgaaggggaagagcttgaggcgctggaggagttgcgaaagatcgaagacaacaagaagcccgaagttccagcacctttgactgcgaagccaggggtcgaggtcaaaggagacgagaataagaatccttctacggctacagcagggcctagcggttccggaatgtcgctcccgccctcgatccaaaagctgagcagcagcgacgacgcggcggtggatgaagtctgcaagacgtacggcatcagcagggagcagttccagcagttgcaacgccgcagcgaggcggcaaagtcgacggcctactgcccctacagcaacttccgcgtcggcgccaccctgctttcaatcgacgacaagaactcgtacataagcggcgccaacgtcgagaacgcatcgtacccagtcggcacgtgtgccgagcgcgtggcccttggcaaggccgtcaccgagggtcaccggcgattcagggccctcgcggtgtccacagacatcactccgccggcgagcccgtgtggcatgtgcaggcaattgtcagtatttctttttgcttaccccccgcttgtgctccgcatccgatcggggattcaatcccggaccagtgatgggatctaggtggataccacacccccgtctggagccccggcgccctttccgggaatttgctgggagtatttgtttatgggaccccaccattgtccagaagatcggcttgctgtttttagttttttttttattgttacaaaactgacctcgccaccctcactccagcatccgggagttttccgacttgcatatgcctatattcatgttcgataaggacaatgactttgtggttatgaagcttgaggctgtaagataccccgccgccaccaacatcggcatgtttggtttttaa

SEQ ID NO: 51 - DNA, 35 bp, synthetic construct; identical to SEQ ID NO: 48
  source 1..35: mol_type = other DNA

SEQ ID NO: 52 - DNA, 35 bp, synthetic construct; identical to SEQ ID NO: 46
  source 1..35: mol_type = other DNA

SEQ ID NO: 53 - DNA, 2393 bp, Pyricularia oryzae
  source 1..2393: mol_type = genomic DNA
atggcgccttcaaccaacaacggtgagctgtaaatgttgccctttggcaatttgatttagtacagaagacgacagttaatatctctgacacgctctaggtcccgattctatccgcatactcgttgccactgataaccatgttggctacaacgagcgtgatcccgtccgccgggatgatagttggaggactttcgatgaagtgatgcagatcgccagagagaaggatgtaaggcttgagattaggccacatgctcatattcagctgctaatgtccatttcccctgatccaggtcgacatggttcttctcggtggtgatctctttcacgataacaagccctcccgaaagtccatgtaccaggttattcgcagtcttcggcaaaattgcttggggatgaagccgtgcgaactcgaattcctgtgtgatgctgcagaggttttcgagggtgcgtttggtcatgtaaactatgaggatccagatataaatatctcgattcctgtcttctctatccatggaaaccacgacgatcccagcggggacggccatttctgctcactcgacctcctacaggctgcagggctggtcaactactttggtcgtgtgcccgaggcagacaatattgaggtcaagccagttttgttgcaaaaaggccgcaccaagttggcgctttttggcatcagcaatgtacgagacgagcgcatgcaccggacgtttcgtgataatcatgtcaagttctttcggccaaaccaggccaaggaggattggttcaatcttctcacagtccaccagaaccaccacgctcacacagccacaagctatcttcccgagaactttctgccagaatggatggaccttgtcgtttggggccatgaacacgagtgtctgatcgatccgatcgagaacccagagactcggtttcacgtcatgcagccgggatcatcagtagcaacttcgctggtcccaggagaagcaaagacaaagcacgttgcagttctcactgtcactggaaaacaatttcaggtcgaaaaggtcccgctgaaaacggtacgaccatttgttaccaaggaaattgtgctatcccaggagcccaagcttaagaagcttgccaaggacaaagataatcgagccaaggttaccgaacaactcatatcaatcgttcaagatatgatcaaggaagctcagggtcagtggttaaaattgcaagcgctagagggcaactcgaccccaggtccagcagaaatgcctctgccacttatccgcctcaaggtcgagcatagcgcgccagacggcggcgaattcaagcttgaaaatccccaaagattttccaatcgctttgccggcaaagtggcgaatacaaacgatgtcatctacttttatcgtaagaagtcgggcgtcggagcaagctccagtaagtggagtgcactgccctgtggcgcttgaacatacactgacagaaaaacaacagaagacaaaaagcccctagcgatccctaatgttatggcagaggatggcaatatagacatcttgaaggtggaggaattggtatccgactatctcgccgcgcagtcagtcaagattttaccacagaagcagatgggtgatgctgtcaaccagtttgtcagcaaggacgacaagcgagcgatggaggacgttgtcattgactccttgactacccaggtcaagggtatgatggcacttgagacagacgaaaacgatgtcgagaaggaaatggctgcacttttcaagaagcaagcgtcaaagtttgaagcgggtcatgggtcaaagaaaagacgcatcaacgtaccgcaaccggatgactatgactcggatatcgaaggcccatgggctactaatcctcgctcagtcatagaacttgacgaagatgaggatgacgaacaagatacagggccggcacccaagtctagtcgtggacgtggcaagggagcctcggctcgacgagagagtgatggggacacgttcatggacgattttgaagacgaggctgagccaccgaggagaacagctccgtcacgggcagcccccaaggcagctgtgccagccaagaaagcgtcggcaaggagcagccgcaagaagggcccctttgaggatagcgatgatgacgacgaagatgcaatggccgttgatgaagaagacgactttgaagaggcccctccacccaaacccaaagcaaagccaactgccccaaaacgggcagtcgcaacacgtagcacggcggcacgtggaaagcagacgactctcaacttttcacagtctcagcgtacaacccaaaagggtaaggggtcaacgcagaagccactggagatcagcgacgacgagatttcagatgatgacggattcgagccaatgctggcaactatgagcaggaaacgttga

SEQ ID NO: 54 - DNA, 35 bp, synthetic construct
  source 1..35: mol_type = other DNA
aaaggcgcgccatggcgccttcaaccaacaacggt

SEQ ID NO: 55 - DNA, 35 bp, synthetic construct
  source 1..35: mol_type = other DNA
aaattaattaatcaacgtttcctgctcatagttgc

SEQ ID NO: 56 - DNA, 2365 bp, Pyricularia oryzae
  source 1..2365: mol_type = genomic DNA
atgttttacagccacgagagtaagccggtttacaagtagctgctcactagttgccctcaacagctcgagctgacagttcaatctgattatatcagtcttgacgagccagaagcatggcgttgctacagtctggtaagatgccgctcacctcgtcacctttcactataaggtgtgaatcccgtaggctaatgcgttcaaattctcagggttcttgctacgctggataggagctgtgccagccgcaaagtatctcgaaaggcaatacaggaagtaaatgtcccaaaggcgtgcgtcaccatcgacgagccgccaggagcacccatcgccctgaggctccaggcaagcctactgtatggcgtatctagagtttatcagcagcaatgccactacgttctgggagatgccgaaaaattccgcatcagcatgcgaggtctgatgcgcgtattggactctggcaccttggatccaaatgctgggagggcgaagtgagtgtgaaaccagttacatcttccaccaaaagtcgctaattcctggtacaattgtaactaacgatgccctcagaaaaaagcagttgatgatccaagacgaccctgagtttcacatcagtaacttttttgacctgcctccgcttgaccttgatgagctaggtaacttgagaccaactgctttcgaatctcagttcaccggcaagtattctcaactttcaccgttttcttcgcagcaacgatcatcgtctggacgcaactcattggccatggattttggtgcggcttccttctttggaagccagtttggccctgacccgtttggaggagacagttctgcccagaaacctcatccgggggcagacatgtttgctcaggatgagctacctctgcgcctggaagattttgacgctggattcaccattgatgccgacgggaacatccacgaacatccagagccggagcaacctcaggcagctgttcctatcgccgcccatcatatgctagatcacccaggtccgcagcaccattcggatgatttcattcctcttatgcttggagatgaagccatccttaaccctggcgatgcgccactgccagacgcagatgccctcccagtcagacagcatgagcaggaccctgattatgcgcagccagaagacgatgctgttgtcactgccgcttcgaggagaaagggacgccgtcggaaggcccttgcgccagatacagccaccgaggtcagcagaaccgaattccgcgactggaccgagaattatgtacagagaatggaggaagagaacaagcgtcacagagcgcgtcgggatcatgtgacaaaggaccaggcagcccagaacgcctataacatcatgtttggtcgtggcataggtggggttggtcaggacatgggccttccaggcttccaacatgagctagctgagcactttgccggccacggccttcagatggcagtttttggccgtatcgtcggagacgacccgcatggtcgacgcaggtcggcttcgcaagctttcggcgacgaagaagattctggatccgaagaaggccggcgtgtccgccctcgatctgacgatggatatgaagcccgtcaaagactctcacaggagagacagctcgaagacgatggcaatggactcaattttggcgactttgatcctctacccgaggtcggccgcgagataggccacccactatcagaccagcatccaccctggcaccgccactccatactacacggatcatcaatgaaaggcagtagcgccaaacctgctgctggtcaaggccctcgccaagttcaagaaagcccgctccaacatcgaggcagggctgtccaagagtttgtgcgatttagcgacaacgatggcctcggattcgatggcagcgctggcatgggctctgtcgatgaccaccctcctgatcaacctgactttcacttccaggaggaccccgcaaatcacaacagctcttctatcagcaccgagggccgcgacttcctttcctacgttcaagcacatgcgcgtgagacaggcaccccgcgtagcaagggagacgagctttgggttgactttgccggcatattccctccaagctcgactgctcgatttaatgcggcatcagcattctaccagctgctgtgcctgtcaaccaaccgcactatcaaggtcgaccaagagggcagagaccgtaacaacatctttccttttgggaaaatcgaggtcggtgtgtgtattgacgctttacaatccgaacaaggcgaggagagtgattatgatctccccagtattggtgatagggcatatcataatgacggcaatgacgacaacgagatgggtaccgaggctgatgccctgcaaacgcactaa

SEQ ID NO: 57 - DNA, 35 bp, synthetic construct
  source 1..35: mol_type = other DNA
aaaggcgcgccatgttttacagccacgagagtaag

SEQ ID NO: 58 - DNA, 35 bp, synthetic construct
  source 1..35: mol_type = other DNA
aaattaattaattagtgcgtttgcagggcatcagc

SEQ ID NO: 59 - DNA, 1996 bp, Pyricularia oryzae
  source 1..1996: mol_type = genomic DNA
atgctcaggcactcggagcgtgtccgcaggccttcgaggcgtctgctgttatcctctgttcctatggaatcccaagttcaagcgaggagtcaaaatgctcgagctagtgacggtcgtcaagaacttaccgggaaatatcaaggttctggtcatccagacgcccaggagagaagcccgagcgctgggtggtttgtggaacacagcaataactgtgtacagcaacaggctatctcccatgctgccagcccgccaccttcgaatgcagacagccagcctgtgactgtgatttcacggattgaagccatcttcgagtcgattgcagccgatatacaacagcgcagggaattgtctatcccgtattgtcgtgtcagaggtactcgtgacagcaatagccagctaagatttccaggacgcagtgtttctgaggcaaggtcgtttggtaagattcctttgctcaaccctcggagacatagtacgtttctgcgggttgtatttaaattgtcctgtttccgtagcccgggtgctatgcgtcctcgagatttcgcatcaggctcttataaccggcaatcttgtgacgaaaaggtgtgtcattaacatcagacgtaaaacaacaaggtacgcctagggatgagttcaggcactaattgctcaccaggaacatattttaccaagccagagatctattccgcgagcaggccgttgttgataggctggtagatgacgttgctttcacactcggagtcgggcgacattcattgaacattgtcggtaatccagatcaatagaagctacctggtggcaatggctaacccatcttgaagaccgccgctggcaagggtctaatcataggtccaatttccttcgtcctcaacggtggcgccagggtctgttgcgacaacgtgcggactgaggtaatcacccccatgaaactctctggaatggattgaatctggagtggccattatgttgattgtaatgcccctctagggaacaattatttgttcaacagaaatactaggccgatttgagtttccgtctgcacgttgggtcttgatcatcgaaaaagaagtgagccgaatacatttgcagaaaccttggtgcctacaacactgacattcaatgcaaggcaacttttaggactcttgcgtcctcccagttctaccggaactcacgtgccggacctggtgttatggttacggcaagttaccgtcccagaacttcagctggcaatggcctcatatggagaatgctctggctaaccatacccttttggttatcatagggaaaagggtatccggacctcagtacgagaaacttggtgtactgtcttcgggaagcacgcccgcggatcccaatctacagccttgtggattatgatcctgacgggatcagaatactgtgcacgtataaatacagcagctctgctttagagcatgagagacaatcggctgtgagcaacatccaatggatagggattcgcttgtcagatatcaaggagcaccatcttagaccatgcaacagcgtcttgcaagatgctggctcccccgtcaacactgaaagtacgtgccatcacagaacaattcgccttcaatgaggaagattttccaagtcaaagaagctgtggccttccgcacgagggtatataatgctgagactagtagcctcttgctaacttaagtgccttgtccgccatgcagtacactcaggattggacgtaggacatgttcggaatcgaccggactttgccatgtcgcgacagaacgctttcgaagcaaacacttcccagctgacaaccagggatcgtaaacttgcacatgagttggtctcaaagctatctggatcattagaaacgaggggagaacatgacaaatatttgcgcgagcttcgagtcatgctcatgctcaatgtcaaggccgagatacaagctgttgacaacctcggggatatcaccgagtggctagacaaaaagctttgctcccagttgacgaatgcatag

SEQ ID NO: 60 - DNA, 35 bp, synthetic construct
  source 1..35: mol_type = other DNA
tttggcgcgccatgctcaggcactcggagcgtgtc

SEQ ID NO: 61 - DNA, 35 bp, synthetic construct
  source 1..35: mol_type = other DNA
cccttaattaactatgcattcgtcaactgggagca

SEQ ID NO: 62 - DNA, 989 bp, Pyricularia oryzae
  source 1..989: mol_type = genomic DNA
atggccatcaagggatacacagttttgcgccggaagtggaagtccaggaagcccatttgggccctgatgttagccgagctgatcaccatgattccactgctcgtcctatttggcatcgcccaacccgataccttccgaacgctcatgtggagaatcggctatgccgagaagctcaactcgaaccccaacatcatcctctacgccctggcaaatcatgagccgattcccaagctgccattcgtttggtcgcaactgtacgtcatcgcgaggttgccccttccttggattgcttgccgatagaaccttaagctctaacatggaagcctttcacagacttaccgagttcaatgtggccatctcagtcatgtcactcttcttcctgctggcgaagatgatcggcttcatcatgaaaatctacttcccggtcattgcggttggctgcaatatcgttatgacggcagtctatgccgttagcgtctacgggcaggccggtcccgactaccttgaccctcggtacccgagcccgacgccttggtatctccggaggagttgcgacgtagccgaggggtatggcgctggcaaaacctgtatgataattcagggtacatttgctgctactgtcgtcatgctgtgagtaacgctttcttttgtttttatgttggctacctggacgacttttggcttctaaggttcgataacgactcaggagactgacctgcctgaaccatagctgcatttacgtgataaacctcggatggtcaatcttcaacatgatacccacaaaacatgacaaaacacacgatgaggatgaggatggagaagagtacgcgtctagcgactcgcccaccgaggtcaagacgtgggagatgcagccacagacagctggtccaggcggtgtaccatttacccctaggacgcaggctttccacaccttagacagaaaattgccattcagggcatacgccgaacagaggcagcagtattcttga

SEQ ID NO: 63 - DNA, 35 bp, synthetic construct
  source 1..35: mol_type = other DNA
aaaggcgcgccatggccatcaagggatacacagtt

SEQ ID NO: 64 - DNA, 35 bp, synthetic construct
  source 1..35: mol_type = other DNA
aaattaattaatcaagaatactgctgcctctgttc

SEQ ID NO: 65 - DNA, 792 bp, Pyricularia oryzae
  source 1..792: mol_type = genomic DNA
atgctgccatcaacaatactcgtgctcgccagcgctgcgctgagcacagcccacacagtcatcacctacccaggctggcgcggcgacaaccttgtcaccaacgagacctacccctatggaatgcaatggatctacccgtgcggcggtatcaacttgacgcaaaacaggacttactggtccaccaagggcggcgccgttgcactccagcccggttggttccagggtcaccagacggcgacgttgtacgtcaatctcggaatcggcaacaaggggcccgatggtggaccactcaacatgtcgctgtcgatggtgcctgcctttggcatctctggcccgagcaagaacccctacccaggcacaatctgtctaccacaagtttcgctgccgcaaggctacacgcctgaggtgggagagaacgccacgatccaagttgtcgagcttgccgtgcacggtgctgctttgttctcggtaagtaatgctcctataataccccctggcgggactaagtatcactggttgtggcatagcctttgactgacacgaagtgcccctggacagtgtgtcgacattacctttgtagaacccgacgacgagcgcctcgaaaaggtgcacgcagacaactgcttcaacagcaccgacattggcttcactgatatctacacaaccaaggtggccaacacgaacatcacctcgacatcagctgccgccgccagcttacggcaacctggaggcctggcatggtatgctggctggattcccatggttggtcttggtgcatgggcattgctgtaa

SEQ ID NO: 66 - DNA, 1425 bp, Pyricularia oryzae
  source 1..1425: mol_type = genomic DNA
atgtctcgcgccaatccaccaagcaactcttcggggtctcgcaagatctcattcaacgtaagcgagcaatacgacatccaggatgtcgtgggcgagggcgcttatggagtcgtttggtaagtacacctctgccggaaccgaacaccgcatcttgcctggacctgctccgcaacatccaaagaatggctgtacaatttggtcaggacggtaacctttcaaactttgcgacttaatggctgacatgaccggctgcgcgttttgctctgttgtagctctgcgatccataagccttcgggccaaaaggttgccataaagaagatcaccccgttcgatcattctatgttctgcctacgaaccctccgcgagatgaagctgctccggtacttcaaccacgagaacatcatttccatcctcgacatccagaagccccgaagctacgagaccttcaacgaggtgtacctgatccaggtccgttgctgctgaacactcctgaaaccgaaacgccgtctactgtacttgccagctaaccgtcatgcgttcgaccaccgtataggagctcatggagactgacatgcaccgtgtcatccgcacccaagacctatccgacgatcactgccagtacttcatctaccagactctgcgtgctctcaaggcaatgcactcggcaaacgtgcttcaccgtgatctgaagccctcgaatctccttctcaacgccaactgtgatttgaaggtttgcgattttggtctggctcgttctgccgcctcgcaagaggacaactcgggtttcatgacagaatacgtcgctacgcgttggtaccgtgctcccgagatcatgttgacctttaaggagtacaccaaggctattgacgtgtggtctgttggctgcattctggctgaaatgctcagcggaaagcctttgttccccggaaaggactgtaagttacaatggcgttcctctgtattgagtgtgctacttgctcccgccccagagtgtgctgcaccgtagacacgatgttctccccagtactgacacttgatactttgttagaccaccaccagctcacgctgattcttgacgttctcggcacacccaccatggaggactactatggtatcaagtcccgccgtgcaagggagtacattcgctcgctgccgttcaagaaaaaggttcctttcaggacactcttccccaagacttcggatctcgccttggacctgttggagaagttgcttgcctttaaccccgtcaagcgcatcaccgtcgaggaagctttgaagcacccttaccttgagccgtaccatgaccccgatgatgaacccaccgcaccgccgattcccgaggagttctttgatttcgataagcacaaggataacctgagcaaagagcagctcaagcagttcatctaccaggaaattatgcggtaa

SEQ ID NO: 67 - DNA, 1713 bp, Pyricularia oryzae
  source 1..1713: mol_type = genomic DNA
atgtcggatctccagggccgcaagatattcaaggtgttcaaccaggactttatcgtggacgaacgttacactgtcaccaaggaactcggtcagggagcctacggtatcgtgtggtacgactttcttctgtcttcatcctccacttttcccgtcgcgcggccgccattctgaaagcccaatggcgcggccttggttgcgcctgtactgcttcctaaagacctgactgacacctgacaccttgctgtttcccactttctagcgccgccgttaataaccagacgtccgagggtgttgccatcaagaaggtcaccaatgttttcagcaagaaaatcctagccaagcgcgccttgcgcgagatcaagcttctgcagcatttccgaggccaccgtaacgtcagtttcgcataattacctgcgcttgatgctgccaatcagccggcgcatatcatgcctggtatagctggacaagtgttgacacgcattcatccgccttagattacatgtctctatgacatggacataccccgcccagataacttcaacgagacctatctctatgaaggtatgcacccgcattacatcaaggataccatagggcaggataccgcagccacagtcttgagccgacaagaaagagcccgtgtatatgaatcttgctaacatcttgaacctccatgtagagctgatggagtgtgatctggctgccattatccgatcaggccagcccttgaccgatgcgcacttccagtctttcatctaccagattctctgcggcctgaagtacatacactcagccaatgtgctgcaccgtgatttgaaacccggaaacttgctcgtcaacgccgattgcgagctgaagatttgcgactttggtcttgcgcgtggtttctcggtggaccctgaggagaacgctggttacatgactgaatatgtggctaccaggtggtaccgtgcacctgagattatgttgagcttccaaagctacacgaaagcgagtacgtatcccctctggcgcgcccctttggttttcaggctaggaagcgcatttgtgtttgcgttggtgtccttgtatccatgactaatattctctacagttgatgtatggtcggttggatgcattttggcagagctgctgggaggcaggcccttcttcaagggtcgcgattacgtcgaccagctcaaccagatccttcatatactcggcacaccgaacgaggagaccctttcgcgaattggttccccgagggcccaggagtacgtccggaacctgccgttcatggccaagaagcctttcccaacactcttcccgaacgccaaccccgatgcgctggaccttctcgatcgcatgctggcgttcgacccctcatcccgtatctcggttgagcaggctctcgagcacccgtatctccacatctggcacgatgcctctgacgaacccgactgcccgaccaccttcaacttcgactttgaggtcgtcgaggacgttggtgagatgcgcaagatgatcctggacgaggtctaccgtttccgtcagcttgtgcgcaccgcccctggtgctggtggccacggtgcaccccacgctccccaggtgccgatccctgcaggtgccggtcaaggtcaatggaaggccgaggacccgcgcccgcaagagtacgtcggtcagatgaatgacctagaggctgagcttgctggcggtttggatcagaggaggtga

SEQ ID NO: 68 - DNA, 2083 bp, Pyricularia oryzae
  source 1..2083: mol_type = genomic DNA
atgcatcttccaacttcattgggtgccttgcatttcttgatggtgctatggttctcgccgcacagtattgcggcactcggctggggaaaccgcgcaaagtcatcgccaccacaaagatcccgcgaggctgcgacgtttcacactgacgcctacgatccgaccttcgtcatccagcctgctgtacttgtcgacgtttacgccgatgccttgcgacaacttcaacagctagagtcggagcctctatgtcatcgcattgccgctcgacttcttgtcaccaactgccagctacttgatggcaaggatgaagccactgtactaaccgacagtgggcgccttatccgcgactttgtggaggcctacgcagcaagtcttgccatctgcgaccttgaacgtggcgatttccacattccttcagcttgttcaccgtttcgagaacatgcacttgcgaaagtctccgctcacagagacctttctctacatgtctcctcgtctcaaatacaagcgtgtatctcaggcctgaaatccccggattcagcgtggggaacgtacatcagctataggcacaaggcgctgcagttttgtgaagcagctagggctgatcaagagaagagtaggttcacttgtgtgttcggaatggaaaggtcctacgactaacatcgacaatctagcccagaacatccttgtgtttcaaaagctcatcaaggtcaccgagcagttggtcacaggggtcgaaaccgagctccaaaaacgtatgaatgatctcgacgagcgaactaaacaagcaagcgatgccatcgaccgcctcaatcccaaactacatggcttacacgagagctttgggaaggttcagatcatgcacaatgggcttagcgaggccctgagggattcacttggcgcgacccgatccgttctagaggattcgaccactttgcaacagcttctcaaagtcatgatagacgcggtcctccaacatcactctgaagtggcctctgccaatgagcaatcagtcgaaagctacgcggccgtcaccgccgccagccaaaggacatcggaggaaatggttcaggtgctctctgcactttcgattgccgcaacatatacggtagagctgaatcagaagctcgtcagttgattgtcttgtctcatcgtttgatatggaagccgctaatattgtggtagcaactctctcgtgtcgaagccgctgagctctcaaagcgtcagaaacttatggcaaacgtaagttttctgttcctcagtcggtatagggcgaaactaacggccaccgccatagggtttggtgcgtctcgagaacataaccgaacagctagttgaaaagtacggcaaacattccgccaagctcgagtctgtccgcaacataaccaatgacattgtcgagacattgaatgacgcccacatattggctaccgctgcgaagaacacgttcacttttgggtcaagtgggtggcttccgtacgtaacattacctctcggatttgttctcgcgggttcctacggtctctcgccgtcactggctcggaacatgttgctggctggtcttagggagggcctagctctgctatggtcgtcccgagattcactctgcatatggccgtccagtttgacgtctttcattttttctacatcttccaacacaccgctcaatgctacgatttaaccactataagcttgctattttgaaggttcacggcacttgctgtgacttgcatctatttaccgggcacacattcggcgcaaacactttttacctcatttctcggacacactctggtacttttcacattctccacttcggcgttttggcacactcacacatatatggggatcaatggtgagcttggggaaaaatgggaccgcatcaagcagcaaagtggctgctccagataatagattatggttactgggcacaggtctctacatggggcgcgataatgagccaacactattgccttcaaatgccgaacatggactcaccgcctctcgttgaatggactttgcttctcgacaaaaaatctcttttcaataaaacagaaactttggctccatttgcattccgggaccgtga

SEQ ID NO: 69 - DNA, 35 bp, synthetic construct
  source 1..35: mol_type = other DNA
aaaggcgcgcctgggcatttgagaatgcatgggaa

SEQ ID NO: 70 - DNA, 35 bp, synthetic construct
  source 1..35: mol_type = other DNA
aaattaattaatcacggtcccggaatgcaaatgga

SEQ ID NO: 71 - DNA, 5327 bp, Pyricularia oryzae
  source 1..5327: mol_type = genomic DNA
atgtccgctccgggccagctggctcggaaccgctccgtctcgagtgcccaaaagtctaggggccgagtcaaccaggactacccagcgatgcagtccaggacgcaggaccgcgctacggtcatgcgatacttcgagccctgcgccgcgacagcatccatgttcctgtatgcgcaaggcagctcggtggtctgctgtcaccacgacactttgacgatagagcggcgattttcgaggcattcggaggagatacagctcttggcggttgatacccagagcgaaacaggggctggacgtttggtggtgagctacgacgcagggcagactgccatagtttgggatctcatgtcaggtgacgaggtggctcgttttgcttcctatgaacaccttacaaccgctgcatggatgcgtaatggcaacgtcgcttttggtaagtcgtcttggtcaatgaatcaagacttgctctataggagcagccgtaatcaaacaattcgtggaagaagaattctgaccgatatgcgcaggcaacacccaaggaaacattatactatttgagccacagacgtcagagcatatttcttcgagaacactggaccaaatagctgtgacatcactagctccgtccgcggattgccggacattcgcaatcgggtaagacgaacaaaggatagatgtgtcattatggatgagctgagctaacaggtatgtcgatatcaggtatcaaaatgggtctctactcattgcaaatcttcagccgaggttcaccattttgcataatctgacaacctcacgaggcccatcgcctattgtaaatctagcctggcatgcctcttcatcgaggcagaaatcagacatgcttgctgtgcaaactaacgatggagaccttcgtatttggagcgtggcaaagtcctacaacaacgccgacccggccaaagttgtgagaattctcaaaaagaccgagaactatctgatcggtccaaattggatggggtggtcaaagaacggaaggataattcagttctctgaaaagtgagccgcccccatttgcagcaagtatgaacattgatatctaccaagaaatggagactgatgatgttttgacagcgagacgttatcttgggacgtccggactaagcacgttacccaggacagcattccatcgttggaacacgtccgaggattagctgtttatggcccaggcgccagtctttttacgttgggtgccaacaataccgtacaacagtttgatctcaacgcacctgcgatgatggtcgccaatgttcagcacccagctaatctgctgccaccatctccgcctgtgtcaatcgaggagcaagaaaaggcagcggccgcgagtaactcggagtcggagatatctatttcgatcgagccaatgacgtccgagagcgaagaggaaaggatgtcaccgctcgcccgcatgattcattctagggacactgcctcgagcggtccggggatcttcaggcctgatagctcacagtcaagccacagtggcacctccgagatttcgtcgaccagctctcaaacgcctgggaggtaccaaccatcagcccattcgcgaggccttacggaaaacacgtatatatctgcagggtcatcaatgttgtcatcggcagcaccacattcttctcggcatcgtgaccgagactcgtactccattggaagcctcagctctgtgtccatggcttcatctagcggccgtccgtcaaaacatcgcccctcacgccttcgaaatgagattccgcgcagcccagaagactcgagggtcgatgatctcttcaaattcactcgaagtcgcctcagcgatatcccttacaaaatgccagccatggcagatgcctcgaggctcaccaatgacgatcttcgacgacagatgttgagcacgattttcggctggaatcgcgaggtagacgacttgattcgagatgaattaagcaggcaccccaactcctcagctaaccgcatcctgctgtcaaaatggctcggcgacatcgagccggacattatcgcaaccagttcagccaacatgacctcttcggattggatgcttctggctctgagcggaatcgggggacaggcatctcagcacaagcttgggcgtgcttacgttcaaagacttcttgagaatggtgacgtacatgcggctgccacaatcatgatcggaatgggcgaccagattgatgcgattgagatttacgtgtcgcacaaacgctacatggaggctctactcctgacctgcctcttcttcccgtcggtctgggaacgccaagcacagattctcaagaagtggggagattgggctgttcagcacggccagcaacaattggccattcggtggcaagttttctccttcgtatttggcttaaccctaaggctatttttatattccccctttgtaaagctactgactgctaacacctgatgttctacttagccttgcctgcataggcaaagaatcttcagagccgtggacttcgccctctgcagcacaactcagtttcggtagcctgaatgccataaactctagcatccctgaggtgctcagtcctccattgtcaccgccaggcatgaacaggggaccgcagcgcagtatcgcaaaggcttcagcgctgaaactcatcacttcctttggagaccaaggcgcaaaggccaagtactttgcaggcgacgatggacagacgcctattgccgcaggcgtgacgcctatcgccgagtctgcaatctcccccggcgcctttgaccctgccaccgctttcatccgtccctcccaacgaagtgccttccccacgcccagctccgcgcgtccttcgaaccaaagctttggtcgacatcgcctgccttcgatcggagaggcgacaggaaagggcgagcagcgtcgacgcacgcccggcccatcgtctcctgtactagaccgtgacggcaaggggcatttgagaggaccgtcatacgattactccaacaacaacttgaacgaggccgaggcgatcggccgtgcagcaactgcaagcccaatgatgatgcgggacagccaccgcaggagagagccgccgcctccatcgccctcgcctgcttcgatggccatgctcatggatcatcagggtgggcgcacgagccgcaacgggccgcgtaatcgcattcctcaaggaattgacttgcaactgcagcccattgagccaccaaatcagagcagtgacgtgacttctcccgagcagtctgtggcctcttcgactagatttcactggccaagccgccggcggggacccggctccgtagccagctcagtcacctctgcaacttccagcgtagcaaaggcacatcgtgcccgaggatatggccaccctggtaaaactctcgatgattatattcacagcatggacaacacggctggcaggcgtgcgaccagccgtggacgcggacgggactcgagcaagaccaggaagtccaagtctcgcgaagcatctcttgaccatgatcagcgtgggcgtgagacttcgagaggatacactccacgagctggcaagcgatctcctcgatcacctgtccccatgtctcctgaggaactaatcaatctcagcaccccaaaaacgaatgatgccagaagagggggcgatggatcagtcattgagattgccacagatcaacccagcaccgtccgaaaattaagcagcagtcagattcggcatgcgtcaaggactcgagcaaacggtggtagccggccttccagccgtggacggcgaacggccagtcccgaaaggatcggtcgcgagcgcagcagtggcaggaatgcatcacctccatctccagtaccaatgtcggccatcccaagagatttctctggctcagaggaggagaatgactatatgagggcgattgaggcaaaggaaaggttccgcaagaagaacactcgtagcagtagccggggtttccgtaacgcctcgccggggtcggcttcccaccggctgatgagcgacaggagaccttccaaggagtctgcaggctttggtgaggctgaggatgccgtcagctcgcttcgcaggatcaaggacgagagacagctcaagaaagaggcagcagctcgagagcttgaggaaagacgcaagtcactggcgcgtagacctgctgcaccgccgatcccacacccggatgagctgtcacctattgttactcgaggcccggccttcttcgagtcggccttgcccagcacggcctttgtgccacccagagatctgcccacacgcagtcgcacggtcgagccgggagagtcaaggagcatgtatgccaaccgtcaaccccttatcgggcttcctgccacacccaaggcgatgcgcttgatcctggaaccagagactggaggtgtgccgggagtccctgaaattcctgtcacctttgcccagagagcctccccaacacagtccaacgcatctccaaggcattcccccgagaaaagtgaggcggtggccagagcggattccgagcagaccaaggcgccccaagagaatcttcttactttactgccctccaccgtctacagccctcccgtgcggccaccaatttctcgttgcatgtcagcgccacccgaggagccgctcgcccccaagactttcaagccttctcagcaatccagctctcgccaggccaatgaccgtaagatgagcacaccggacgtgtcttcggaccttcgccaggcgggcaacatgaggacaatagacgacatgctggcaaacaacacccaaaggccgacgcatgagtcccaagggatgccacctcctcctccaccccctccagtgctcaaagaactgcagcatcttgccatacccccaccgccgcctcctgcgccactttcattcagccaaaagtcgcagcaacctcaagtctatggagggcgtaccgctggaatgatcgagatagtgatggacaatgatgaccagatccctcctccaccccctcccccgccgccaatgaccatgtcggcgccgccggttcctgtggctatcccagtaagcgaggccaccgttcctatcctctcgccaccggcaccgccaacgcctaagtccaaccaccagcggggtcgcagcagcatcgacaacagcatctcgtcgcgcatctctcgtgtcaccgatcgcgttcgatccgccagccgtagccggaccaactcttcgatgctctcgcgcaagtcgcccgagcttgcgaaccaaacctccccatacgagagcattgggccgcccgtcagcttctctgcccgcgctgtggctcaggtccagcagcagcagcgcactcagactggtcttcagcccagtgagatgttttga

SEQ ID NO: 72 - DNA, 35 bp, synthetic construct
  source 1..35: mol_type = other DNA
aaaggcgcgccatgtccgctccgggccagctggct

SEQ ID NO: 73 - DNA, 35 bp, synthetic construct
  source 1..35: mol_type = other DNA
aaattaattaatcaaaacatctcactgggctgaag

SEQ ID NO: 74 - DNA, 2816 bp, Pyricularia oryzae
  source 1..2816: mol_type = genomic DNA
atggccatgttggcttcaaagtcgccttttccggcccctctggccacttcaggctcaggaatgatggctgggacagcacaagcatcataccctccctcgagacgagcaccagctgttccgcctgccagccagtctttcagtccgaccgagtccgagttctccgacagcgatgatcatgattcaccaaagcactgggacgaagacaaggtctgtgaatacctgaggagcgttcgctgtggcgagtacgagaagctcttcaggaagaaccatatcaatggcgagaacctccttgagatggacaaggatgtcctcaaggagatgggcattgagaaggttggcgaccgggtacgcttgttcctcagcattaagaagctgaggacaaaggccatcgccggccagaagaagaggaatagagtgagtcgggggaatgcttcctttgcggctcgaaacgcaatggctgactttagttaccgcttcaccaggattcctttgccggacacgagagcatgtacactccagtatctgaatctcccagcaagccctttcactctagcagccgtgtcatgcccaatccttcagtgaacaagagatactcccgtcagattgacttgagcggcatggcatatgatccctccaggccgaccacttcctccaggccaacatcgccgcttcccagtgccgatttccggactgcgcgcacacgaaacccatatgttggacagcaacccactcctactgggtcgctgagaggacttggatcaccaccagatagccaggcaaactcacgtccggtattaacccatacccggaccgattccggtatggacggatcgctgatggctgccttaccacagaaccaagatgtcattcgtgtcatctctacagggggcgtcaccaaggttgtcaagattgccgactgcaacacgtgtgaggaggtgatgcgggtaacattgcgcaaattcgcgctgcgggaggaccacgagaggaattattgcttctgggttctttctggacttgacccagatccgaagcagtgccgtagactgggagacaccgagctttggcgcgtcattaaagaccagaagcgcccggagcgcaaccgacttattcttcgtcgggtaccggctggcgagccaggacagtctgagcttgagagggccgccgcgattgccatggaggaggctcaacaatcgcactcccgcgccatggacaacgttggggcgcgtagccagatcaaggtgcaaaaggttctcggagagaattgggataacctacagcccccgctctctcccgtcttgtaccaggatcgcgagagaaacgtttacaatgctgctcgtgacctagagagacccgaacctctggattccggccggctgcagcctaggagaaaggtcttgaggtcttttggcggtctcaggcctccgagtgaactcattgcttccgacctgaccacttacttccccgaccacccgcgggaggacattgatcggactgcgagactgtctatgcgtaggtctgcacgccttagcaaggttaacagccgccttagcgttgccagcagttttagcatggcctcgagcattcaggatgctcctcccatccctaccatcgccgacagctggctacagtcgacacccttacccaaggctcgcccccgagacctgcagagtaggctgcagcatggctaccgtgattcggtggcgtcgtctatgctagacacgcttcaggaggaagggtctcctatagaaccgaaccgcaagtcctatgtttcattcgccgacagcggctcagattctgctgccgtgagtgtcacggaccccgacggaaacattgtccgccacagctatttcgacgagggtagcaccattggttctggctctggctccggctcgttcggcgatgtcagcaaagctctgaacgaggatggagaggacgccgacgaagatctgcagagctttctctctggcgagtcttgggatgacagcaaatggatgaagggagcactcatcggacagggatcctttggatgtgtctacctcgctctccatgctattacaggcgagctcctcgccgtcaaacaagtcgaggccccatcgcctggtgccaacagccagaacgacgccaggaagaagagcatgattgaggcccttaagcgtgagatcagcttgcttagggatcttcgccaccccaatattgtgcagtacctcggctgtggctcttctgctgaatacctcaacatttttctcgagtatgtccctggtggctcggtccagaccatgctcaactcctatggcgcattgccagagcctctggtccgcagttttgtgagacaaattctgaacggtttgtcgtatctccacgaacgtgagatcatccaccgagacatcaagggtgccaacatccttgtggataacaagggcaccatcaagatctcggactttggtatttcaaagaagatcgaggccaccaacctcctcaacggcgccaacaacaacaaacaccggccctcgctgcagggttcggtgttttggatggcccccgaggttgtcaagcagacaagttatacccgcaaggccgacatctggtcacttggctgcctggtcgtcgaaatgatgacgggtacacacccattcccggactgcacacagctgcaggccatcttcaagatcggtggaggcaaggcaacgccgaccattcccgaggatgcgagcacagaggccaaggctttcctggcccagacttttgagatggatcataacaagcgccccagcgcagatgacctcatgctcagccccttcctgactcctatcacgtaa

SEQ ID NO: 75 - DNA, 35 bp, synthetic construct
  source 1..35: mol_type = other DNA
aaaggcgcgccatggccatgttggcttcaaagtcg

SEQ ID NO: 76 - DNA, 35 bp, synthetic construct
  source 1..35: mol_type = other DNA
aaattaattaattacgtgataggagtcaggaaggg

SEQ ID NO: 77 - DNA, 1099 bp, Pyricularia oryzae
  source 1..1099: mol_type = genomic DNA
atggctgccgcaggaggagcgtcgagtattattactcaggtgcaacagggtggaccgccaatcaactcgatcggaggtatgtgagactgcggctcggagtaacgggatctggctttctaatgtgtgcatgaactaactgggtcatagatgtcggcgctgatgagacgatcacgatggaccttcggggcacgaggttctccctctcccgtgatgaactgttgacattgcccgaattcgtcctgctttcgttgtttcctaatggcttgttcccagaaggccacatgggcgggtttgctgacggtgatgccgtccaagtcgatgtacgtggagactgggtttctatccttcctatcttttaattccgatgcctctagttcacctactaacttgattacgaacagtacgacccggcatctctgcagtacatgctggattttttccgtaacgtggcacagaccatacctgcagactctgaggtagacaacgatatggtgccggtcgagcctatgggtagcagcagggacgactcatccaagagagcaggaatcattgtgctccgtgaggacctagatttctatgccatcccgccacggcctgatatcaagcagccagacatgatcgaggtcaagcgggccgcggccagggcgctgctcaagcagaacggtatcttcagtggccttaagcggagcgatgagcctggtacgaccgaagcgcatctgatcgagatgttgactgctgggtaggtccccctttggttttaggacatatgagtggactgttttgtgtgctaacaggctggtgtttgacttccagtggctttgatcacgatgacaaatggggccacagagccggagagcccaataaggcagtcatttgcagtctcgcgctggcacggctacgcagcgacatccgtggtaacgaaatgggtagcaatgcggtcggcatggcacaaaagttgttgttgttctggcgcaagccagcacgcaggtgctggtgggagggtgtagagcttgacaacgtggagggcgtcgaagggaagctcaaggtttggattcgtcgggtgtggacgcttgagatgagcgtcatcggcctgcgctaa

SEQ ID NO: 78 - DNA, 35 bp, synthetic construct
  source 1..35: mol_type = other DNA
aaaggcgcgccatggctgccgcaggaggagcgtcg

SEQ ID NO: 79 - DNA, 35 bp, synthetic construct
  source 1..35: mol_type = other DNA
aaattaattaattagcgcaggccgatgacgctcat

SEQ ID NO: 80 - DNA, 3910 bp, Pyricularia oryzae
  source 1..3910: mol_type = genomic DNA
atggagccaaatagatcaaggggcttttcggatgaagagctcttcatgagtcgcccggtcgacgactgtggcgacagcccaaccgtcgagccccttcgcatcttcaacaagagtcctgccgcctcggatcaggcccgtttcaagtacccgcgacccccggagccggcctcatcggcttcgccctcccacaagccaacgttcccgctgccccctggcgcatcgagctctgcggcgcccctcccataccccgacgatgaggatctgcgcccttcgaagccgctccaatccaggctgccttacccagacgatgatgttggtcggaggccttcgcccgctggaaggatacagaccagcagtcctgcaagctctggaggaagctacaatgacacatctccgcgcctgagcctcagccccactggcgaaaagagaccaggtcttgctgaaaggaggggcaccgcgcccagtgcgctgtcgccaacaagtccagatggggacaaggataatctgttcgcgaagcctatcaagccgcccaagcagcaacagccacaaccgcaggagccgcagcctaggatctcaaacagctaccagagcaaaccatactaccctccgcctggaggcagctccgcaaacaatgctcagcggccgactgtggctacaaacacgctcaagatgcctcaggaaagcagcgtgaaccgtttcaactcgaatgcctccacgtcaaccacccgcgccagtcgcggctcacctccgcctccagaaaccccgatagtcgaaccgggtgtgattcctggtggtggcatagaggctcgctatgctgcctcgggcatatctgggaccgcgaccctcacggccctccaagcgcaacaggcgcagagcgccgcggcctcgcagcgacttgcccagtatggtggacagcccccggcacaacgcccgtggacgccgacagagactccggaccaacagccccatgggcccccgacggtttaccagggctcaaatccagtgggaagcccgtctcagtcgtccacggcacagaacggacaatcccagcagccaagtttgcaagttagcgttctggagcaggatttccagcgcatgcaagcttcaacccctccccctgcatactctagcgtcagtggaggtggtaccgggtatccaaacgagaaacagcgccctgcgttgcagcaacagtccagttccagctcgcaacctgggcaagcgcctgtcgctgcaagttctgcggccgccactacatcggcttcagttgctggatccagctcttccggcgcagttcagactcccgttgctcaaggcccggagaagaagccgcaacagcagcagattccaaatcacctggcttcgccggctctacagcatccgggtcatcctgcctttgccaatgaccccaggccaggaagctcccagaatggccaaccgaccatcacacacacgccatcggttttacattctcagggcccctcgtcgccacccccactgccagaaggatggatctcccatctcgaccagaactctgggcagtactactatatccatcttgccactcaggctacgcagtgggagttccccaagggtccaaatccgatcaaccacgaggtagccccattgtcaccaacagcttcgacttatggcaactctcttggttctcctttcctgagtggtaaacagggaatggcatcgcccggcctgtatcctccccacactcctggctacgctgagagtattatgagcgtggcggcctcggctgcacccagtgctgctggcttcactggacctccccccagctccggcgtggagatcttcaaggttgcccctacaaatggtgtttactttggcccctacttgcggtacgtcaacatggacgtggagaggggtgtgtggttggggagcataatgattgtcacggacgctcctcagccgcccacgatacacattcatcgcagtgtagacttgtcaccgaacccgcggcagctcatgccacatgtgattcatacccatcaacgctggagcttttacaagtacgacttggatctgcaaatgggcgagcaaactgagaaatggacttatgcggtcacgtcccacatgggatgtacgcgttacgagttcgtcgttgcggggcgcagtgaaaccggctggcgcttcgtggcgcactcgggtaacgattttgcctcttcaacttcgcaaggcgacagggcaaaactcggtggcgtcggcttcatgtggaaggacgtgctgcaaaggaatctggagtgcggcggttttcacgtacagctggggctcggtgatcaaatatacggtgatcggctctggaaggaggtgcctctgctaaagcaatggctcgccatccaaggaagggagaatcgcaagaccgtgcaatggactgcgcggcatgaagaagacgtcactcatgcctacttccactattacacgtcccactttgaccagccattcttgagagaggcgtttgctcagatccctcacatcttacaactcgacgatcacgatatgtaagtctattttgtcttgaaccccctatcgtataagtttgattccgctgctaacacgactccctcgtcaccaacagttttgatggcttcgggtcttatcctgactacatgcaatcttcacaaattttcaagaacatcgggcgtgtggccattgaaatgtacttgttgtttcaacaccatacgactgttgaaatattgcgcaatgttaactcggacattgatctgttcactataacgggctctgggtggcactttgtcaagtacttgggcccggcaatggtcgtggtgggtgttgatatgagatcagagcggacccaaacgagagtcttggccggtccaacgtatcaaggcatctttccaaaggtcgccatgttaccacccagtgtccagcactgcatctttatgctatccgttccgcctatctatcccaggctcgacacggtggagagcttggcaaacacattcaacacgggcaagaaggcggtcaactcgacatacaacctgctcggcaaagtgaccagctcagtggcgggtgtagtcggtggtaaggaggtggtgcagcacggcttcactcacgtcaagaaggcggtcggaaaaactggtctcatgggcaatgttctcaaccagtttggagagtttgacattggtgaggaactcaaggacctgtggacgcatgagacgaaagacttggagcggacatacctgatccggactctgcaaggaatttcccagcagaagggaataaggatgagttttctttcaggaggtgagtttctttccatgtcttgttcctggaaacccctgccctattaaatatccagtccttctgggcgcggcataagttgcaagcccaaaataaaaaggtgactaagctgaccatgatatgaacagatgtcaattgctgcggcgccgggttggttcacgacccgtctcaccctagcgaccacaagaccatgtaccaaattatcacctccccaatcgtggcggcaccatcgggtaactacatcctcaagatgcttcacaactccaataagatgctttatgtgcctaccaacggacacaaatccaatggagaggtgtcggacaccaaggaggacatgatggagatcttccaggtcgacgcgaatgggtcccaacgcgagctcaagaagcttatgggacgtcgcaactatgttgctgttgtggcgtacgaccccgaagtcatcaacgccgcggcaggatcgcagtacgccgcaagcatcatgaatggcggccaacctcagggccaggggctgcagaagctcagtcttgccgtcgactttgtggttcagggtgacggatcattcaatacgcccacgaccaagtacggacctgtcattatcccacacttggaatatgggcactga

SEQ ID NO: 81 - DNA, 35 bp, synthetic construct
  source 1..35: mol_type = other DNA
catacacaaccgtcggcgcgccatggagccaaata

SEQ ID NO: 82 - DNA, 35 bp, synthetic construct
  source 1..35: mol_type = other DNA
ggattgattgtttaattaatcagtgcccatattcc

SEQ ID NO: 83 - DNA, 2223 bp, Pyricularia oryzae
  source 1..2223: mol_type = genomic DNA
atgtcaacaatatcccccaaccttcaggccaacctcgcgacagcatggccagtaccaaaaatggctgtcgcatcagcaacaaagacaaagccggccaaggccgcggccgccactgccaatggcacttccaacaaaaagagccagatgcaccgccgttcgagaacaggttggtaaccctcctagcgtgccttaaaatctctcacacaccggacttagaccagactatacttttttttttttttttgcgattcacgctatgaacctctataaactaactgtcaaccacccccacttacaggctgctacacctgcagattaaggaggaaaaagtgtgatgagggtcaacatgtttgctcagcatgcaagcacctcggtctcgtatgcgaatacaagcgcccgcattggtggagcaacaacgaggccaggaggagacacaaggatgatatcaagacaatcatcaagaagaagaagctcgccgagaagggtgcccacgctgtccaaaccggcatgagctcacccccgggcctgtctcactccatcccgtcgctgccaacctcggccaccttctcagaccctctcgacaggacacgatccgcctccatcgactcgcactttagcttcaacttcaacagcccgccaacgacatgctcagaatatggtgcattcactcctcagctacaccccgacttcatgttcaccggaccatatgcttcgccctacgagatcgacgtcaagactgagaggcaaatgtttgttaatgatgtgcctaccctcagggaatcaacaacctcgacctttagcacctgctacaccccgccgccaccgggcacaaccctgccttcgttccctctggaaggtgaatggactgaacaggtgtgctcggaacggcgggagtccttcaccgaggagactctgaatgtcaacttctttgattttgcccatggccgctcgatgcagtcaaggcaagttgccattgagcttgacgagggtgaccaacgcctgctggaccattttgtccgacatgtcctgccgactatcttccctatcctggagtccaaccagcacggctcggtcagctcagacctgatcctgccggcgctccagagcaacaagggttatcttcactgctgcttgagcatcgccgctcaacacctcaaggctgcaaccggctctcagagcgaggacatggatgccgacatcatgcgacaccgctacgcgaccatctctgcgctttgcgacgctctgaaccgcgacgagaaccatcaacagattctcgaggccgcgcttggcttgatcttcttccagtgcggcgtcgggcgcttcgacgatgcccttccagacattgcgtggcatcaacacttccaggccgccatctctcttgtgcagaagcttgaccttccccgcattgtctcagaccccaacgcagaggctgcaccaacaccattcaacatgactctcactgcttggatcgacatcctcggtgctacaatgcagggccgcgcacccaccttcgcccacacctaccgtgagaagcatttgtctgcgaccaactcgtctctggggcttcgcgagctcatgggatgcgaagaccgcgttatgtacctcatctccgagattgcctgtctcgaggcactcaggaatgacggaatggacgacatcactctttgccaacacgttcatgttcttggtgaccaaattggtctcaccgaggttggcgagactgcccctaagctgccgttcaactctaatggttcgctgagcccaaagcagttgagcaaaaacatcacggcggcattcagactcgcggcgcgcatctacctgtgcagccttgtgcccggcttcaaccctacacaggctagctgcatcggcctggtcgaaaagctgaccaacgttctccagcacatcccctcaggccaccaaggatttgaccgctctcttgtgtgggtttacctggttggcgggtccgtcagccagcccggctcgtctttccgtggcttcttcgaggaccgcgtggcacaactcggtgaggcagccaactttggctcctttggccgcgtcagctcgctgctgcgagagacgtggactgaggccgaccagctcgtggccatgcagtctcaggcttgctcccctgctgcatcggagacagggagcgtgatccccacacactacatccactggagagatgtcatgcagacaaagggctgggattaccttctcgtataa

SEQ ID NO: 84 - DNA, 35 bp, synthetic construct
  source 1..35: mol_type = other DNA
tttggcgcgccatgtcaacaatatcccccaacctt

SEQ ID NO: 85 - DNA, 35 bp, synthetic construct
  source 1..35: mol_type = other DNA
aaattaattattatacgagaaggtaatcccagccc

SEQ ID NO: 86 - DNA, 1425 bp, Pyricularia oryzae; identical to SEQ ID NO: 66
  source 1..1425: mol_type = genomic DNA

SEQ ID NO: 87 - DNA, 35 bp, synthetic construct
  source 1..35: mol_type = other DNA
aaaggcgcgccatgtctcgcgccaatccaccaagc

SEQ ID NO: 88 - DNA, 35 bp, synthetic construct
  source 1..35: mol_type = other DNA
aaattaattaattaccgcataatttcctggtagat

SEQ ID NO: 89 - DNA, 4666 bp, Pyricularia grisea
  source 1..4666: mol_type = genomic DNA
catctgccaagctcagctttcacttacaccgagcatgggagagacgcaagggatgaagtccattccaaaagaaacccgccaaatcgcttcccataaagctttctttgtctcaaagccccaccaatctcgcttggacctccataccaacttttgaaatctttcctctttcatactttcatatcaccctttcgtgcacacatttagcattcaatctgcttgaagctgcaatacaacggcatttcaaaacgacgcgatggcgcctccctcaagtgcttccaatggagacaagattcggcaaatgattgccagtctctcgcctgacgacatcgccaggctgattccccaggagactctgacttctctgctcagagcaaatgacgagaaagagcgcctgcgggagctgcccgttagcccgagagcggtagcagcggcgagcaaaaacaagaagaaagtcaatggatttatggcatttcgatgtgagtacagactgataatagagaaatcgaagcttgtgctgacagcagtatagcctactacgctggcatctttcaggatagaccgcagaaagaacgttcgcccttcatcactctactctggcagaaggaaacgctcaagtcaagatggactctcatggccaatgttttctctcgcattagggactttgcaggcaccacaagaggtcgtatggcaatgagtggattcctgcgagttgcctgcccgcttctgggcatcaccaaaccctgcgactacctcagacgctacaattgggaactcgagtttgttgcagacgcgtcagctccgtatgatgctgctatgaaatacgagatttcccagtcacaaatccctcacattgtcgacgaattcgaggtccctactacggagattgagttgcttcgcgcctgcgttcagggtggctttccatttgagaacagtgcccagcttctaagagacatggaagacagctctgtcaccgttatgaccagaactgcgcctatcatggcaccctcgcatgcttcgcaggcctcgcatggccaacataaccaccatttcatcaacacactcatcaacgacccggatgctgcgatatctgcgcttttgccccaagatgaagacattggcagtctgatggttgacatgaatatcatccactcactcgagacagacagctcaacaacatcatcggcacgcaactcagtttctcctctggagcagcacttgttctttcacgaagacgtctccatcgatccttcaacaatggtttctttccctggcgaaggtcatggtcacccggaaacacaatacagctaccccaatccaacgctaggtctctggtaaatcagaccatctcaggagctcattttagtctagtttttattgagagacaggtcattagttgtcacataataattctcgcttgcatctggtcattttattaaaggcaggctcatcaaattagcgggtgttttttcttcaaatatcaacgacgagacaaattcaaccattccagaacaaaagcttcttaattcagtcggagcaatcattctgtgagaatgctggtgaataagtattttagcctactgataggcacggtacgtccactctcgatgagtctgcatacccgtcacaatccccaacgaccaagccaagtcccctgaagcccgcagaaagtgagagagaaaaacaaaggtaagagttcccttatggtcgtaagcaggtatctcctaagtatcggaggttagatgagcttgaccagagaatatggatacaagttgaaacttaccccaagtgtacctaaggcaagaccatgcatttgatagtagttgaaggtatgagctacacagttctgttaaatattagtaatgttttagtttctcaaaatagaagagtcaacaagcctaccactggaggatttagaggtagccgcgcgcgatcatttgcaatctttatcttgggtcttctcaaagttagcagtgtaaatacagggacatgttagagtgcatacctgctcatcttcatagctcaagcgtatgacgctttcacgcagtgtagcagcttgctgacgtgcggtagtgtagcaccccattgtagaacgtatcaaggagttggcgcagtgagttgttatgaaagtaaaatcgcgcagcttttcttgatcgaagaaaggcaggtctaggacccgatgaaacaggccccatcggctgcccggcattgttggaagagaggggtgctcgataatatcaagccattgcccgtagtccttaggatgactgtgctctctgagaacaaggcaaccatcttggaccctgagaaggccaatagaagcgctgacagactgagcaactggctcatactggagtgtccgcaccctcattgccagaagggtcaccacggcggccagaagacaggtattgcctgagttaaccttggttcgctgagataaatcgaagcaaagcgaaatagcatagctgagctttcgggcgtgatctgaatcacgtatggcgcatcgggctcggtgtaaagcaccctgcaggctctgctctgtccacttctttggaagaggctcagagccgtctttgtaagccttcagtgtgtctaataatgcttgcagggtaaaaaactctttggttgcttgcaaagcagagacaatggcttgatggcactcggtgttttggttcatgctgctatcgcctaagagttccgcgacagaaccgagaagggtcttgcatgcagatacaaacgggcgcgctcgatagacagcaatatcctctggctctggttttccattcttgtagaagttgaagggaggaatctttatgtatagataatctgatgcagttgacattacgccgttgacgcgacagtcatggatttccttggctatttcgacaggtctccgggaagctgctggagtctaagagcagtaagattgggtatggcaaatcgcttcagcagatgagcctcaggtgagaaacgaaatcaacaatcgacaacctggcccgtgggtctgaacaatagtaagcccacaatcaatacacaataccaaactgccatctgctccactccacgctccacatattggtattgttcttcaacactccacctcacaatagcaacgatactactattatgccctccaatctcgaaaaactataaatacttcccttctctccctcctctcgacagatcttcaactctctctctctctctctctctctctctctctctctctctctctctctctctctctctctctctctctctctctctctctctctcttccacatcaaacagctcttcccaaaaaacttcacttacagcaaatatcacaaactggtatctcatcgtctcacgcaatggactacgagaacagcatagtggcgagccagatgcctgcagagaggatatctgtcagcgtctcgatacctcaacaaacagttgatttcgaggtgccggccctctggtcgctaggcaaagtttgcggcatcgcttcggagctcaggtaagccgacccagagtcctcacaccagagcgacagctcttcagcatctaagcgatcacaggctaacacttttggcgcctcaattagcaagaacatggcctgcatggtttggatctgggtcgtctgcgttcctcagaagcggtaccgcatcacgacagctcgctggaactccagtgggctgctggttggccgcgttgatcgtgagttttctactttcttcaccttttccttccctcccagatctgagcagagactgacaagcgacacaaaacctccccacagctcctcctcaatctgccaccacagcgtcctcacagtcatcgtcattcgacggcagtgaggaagacacaaacacaaacatcaacgccaatggtatcgatgagaacctgctgccgcctgctctccgcggccgcactggaccttccaagcctccaaaccgctggattctctaccgtgccgccaagtcagctgagctgcgggcagacaacccatccatgaacgcgagcgaaatctgtaagttcttcgctcttttcactctttttctccgctaccacttgtacctaccttttccccatctcccatactctttgaaaagtctccagtcccacctctcaagctgctgttttgacaagataaaagactaaccaacatctctctcctcacacagctcaagttgcatccctgatgtggcaggcagagtccgccgcgacaaaggcagagtgggaggagcgcgcagccgaagcccgcgaggagcacatgcgaaacactccagagtatgcggtggcggccggtctgcgccagcgcgccatcgccgagaggagaaggcagaggcagcagaagaagaagcaacaggagcagcagaagggcgacggtgacaaggtggccaaggagacttctacatccacagagagcttggtcactacggacgtcggcgctgtcagcaaccacggcagcagcagcagtgaggtgcctgtcacaagcccacactcgccgacactactcagtcccgcgtctgacagcgattgtacgcccgtcggcagccctcgagctcgccacggctggggttctgatgctctcagcctgatgctcgacgccgccgaattctctactctcttctgatctggtctctggcactctgagcgtgctattcccaggaaatcaaacacacaa

SEQ ID NO: 90 - DNA, 3237 bp, Pyricularia grisea
  source 1..3237: mol_type = genomic DNA
tctcattttctattcaggtttattaagttattgaggaaccaactggggaccccacttcgtttctttattaactcgaccttcgaacccaggaacccaactccctccaagactccgacatcaccaaaaccacaagactctttccattcgattgcgctagaactactcacaaacctcagattgcaaacacaaaccccatcgtcagatcattgaaacgaggcacatctacaatggattcattgcagatggactcctctcaaatggaggcgttgtcgtcgatttgggtcatcgtgcagcatcagctcgcccaaatcaacaattccaacaacatagctcatatcggcgccgttctcctcaaccaacttgaggcgcctttcaggagcactttgacatcatggtttcagcagtaagttctccataagctcaaggcttttccgcaagggaaactaacatcaggtaggcacaccggcatcaaccaggtctcagtcgtgcgcgacatcaaggctcgtcgacactacatcggaccaactgatgcttttcaggagagctatcaagttgtacacatccagggtcacggatttgtctggctttgggatctccaggttgatggtgaggatgccagcatcaattcctgcaatatctctgccgagacagcacagaacttttcccagctgcgtcttgacgagatggcgcctaccaatgatgttacgatggtaggtgatgagagcctcatcaacggcaacggcattgactttgccatgttggaagacatcggaagccccgcatcaaacggctcctcattcccgagccctcaagttttcacccgggaaatttcattcgatgatctaccagttggcattatgactgccgaggccattcagagagaccttcttggcgccaatattcgcccggctaacctcattgatccgagtcttgcgagcaatcagaatgtccacaacatcatccatcagaataacattgcccaggcttttacagatcacctgaacatgatggcatccaatgctgtccacgatgacacagaagagggtctgacagccgcggatcttatgccggcgttgcatcgcatgttcgtgccgggtcttgagtcaattgcaatggagcagttccacaccacgcttcctaatggcgcactccttcacctgtcaattcctgtcgatgaacctgaggatgctgtctcgaccaccgcgcctgctgctcaacagacttccttgcaagacaagatccctcgtcctgcgaatgcctacatcctgtaccgcaaggattggcatcccatagtcaagtctgcaaatccaggaatccataacaacgaaatctgtgagttcttttacctccaaacttccctagctgctgctaactttttttcctttagcaaaaatcctggggaagcagtgggcagctgagacaccggaagtgcgggctgagtacaaggagctcgcggaggagaagaagagagagttctacgcaaagtaccctacatatcgctactctcctcgtcggccgagtgagataatgcgccgagtgagtttgtaacacattattgcgtgaaagagtggacagcgagctaacaaattacttgccaacaagaacacgaaaagccgaaagaccccaacgaacggggcagcgaagccgagcaaagcaaagaagtgcggcaacggggttactggtggagcagacagtgcagtcgatgtcagctcccggggatcgccattttagatgaggtcaccattcacatcatccgagatacattgtacaagtcaggagcagttatcaaagctgcatttcaccagagtcctcatatctgattttttcttctttcttttcacattgccccatcgtacatccagagagctggactcgaaataccctctcaatagagtctgcaaagaagatcttaggacctacgacataggttacgtggtcattattcaccaagaactacatatctgccagcgaaacatattcagttttcagagccatttgtcgaaagaaattttgagatgccggccctctggtcaccagtcaaagtttgcggcatcgtttcggagctcaggtaagccgacccagagtcctcacaccagagcgacagctcttcagcatctaacgatcacaggctaacacttttggcgcctcaattagcaagaacatggcctgcatggtttggatctgggtcgtctgcgttcctcagaagcggtaccgcatcacgacagctcgctggaactccagtgggctgctggttggccgcgttgattgtgagttttctactttcttcaccttttccttccgtcccagatctgagcagagactgacaagcgacacaaaacctccccacagctcctcctcaatctgccaccacagcgtcctcacagtcatcgtcattcgacggcagtgaggaagacacaaacacaaacatcaacgccaatggtatcgatgagagcctgctgccgcctgctctccgcggccgcactggaccttccaagcctccaaaccgctggattctctaccgtgccgccaagtcagctgagctgcgggcagacaacccatccatgaacgcgagcgaaatctgtaagttcttcgctcttttcactctttttctccgctaccacttgtacctaccttttccccatctcccatactctttgaaaagtctccagtcccacctctcaagctgctgttttgacaagataaaagactaaccaacatctctctcctcacacagctcaagttgcatccctgatgtggcaggcagagtccgccgcgacaaaggcagagtgggaggagcgcgcagccgaagcccgcgaggagcacatgcgaaacactccagagtatgcggtggcggccggtctgcgccagcgcgccatcgccgagaggagaaggcagaggcagcagaagaagaagcaacaggagcagcagaagggcgacggtgacaaggtggccaaggagacttctacatccacagagagcttggtcactacggacgtcggcgctgtcagcaaccacggcagcagcagcagtgaggtgcctgtcacaagcccacactcgccgacactactcagtcccgcgtctgacagcgattgtacgcccgtcggcagccctcgagctcgccacggctggggttctgatgctctcagcctgatgctcgacgccgccgaattctctactctcttctgatctggtctctggcactctgagcgtgctattcccaggaaatcaaacacacaa

SEQ ID NO: 91 - DNA, 2024 bp, Pyricularia grisea
  source 1..2024: mol_type = genomic DNA
atgatgctcaggcgctcggggcgtgtccgcaagcctccgaggtggctgctgctgtcctctgttcccgtggaaccccaagatcaagcgaacagtcaaaatactcgagctagtgagaatcgtcaagagcttgccatgcaagatcaaggttctgatagccgatattctcgggacagaagccagagcgctgagcggtttgtggaacacggcaatgaatatgtacagcaacaggctatcatccatactgccagccggtcacctagcaatgcagagagccatcctgtgactgtgatctcgcagattgaagccatcttcgagtcgattgcagtcgatatacagcagggcagggaattaactattccgtattgtcgtgtcagaggcacacgtgacatcaacagccggctaagatttccaggacgcagtgtttctgaggcaaggtcgtttggtaagattcctttgcccaccccggggaagcggcaaattacatttctgcgagctgtatttaaattatcatatttctgtagcccgggtactgtgcattctggagatgtcacaccaggctctcataagtggcaatattgtaacaaaaaggtgtgttaataacatcggatgtagttctttttggctgacgcgaaaccaacaaggtacgcagagggatggatacacttactaattgcgcaccaggaacatattttaccaagccaaagctctattccgcgaccaagctgttgttgatcgactggtagatgatgtggcattcacactcggagttgggcgacattcattgaacattgtcagtcgcccagagcagtagcagtagcagtatctgatggcaacggctgacccatctgaagaccgccgctggcaagggtctggtcatagggccaatttcctttgtcctcaatgatggcacgatggtctcttgcgaccacatgcggactgaggtaatcaccccgataacatactcctgaatggattgcttctggtcttgtcatcaaattgattggaatacttatccagggaacaattatttgctcaacagaaggactaggtcaaattgagttcccttccgcatgttgggtcttgattatcgagaaagaagtgagcggaatacatctgcagaaatattggtgctcacaacactgacattcgttttgcaaggcaactttcaggactcttgcgtcttcccagttcttcaggaactcgcgcgccgggccgggtatcatgatcacagcaagtcaccgccctaaaagtttggctggcatagcctcaactgagggacggtctggctaatcacaaccttttgatcgtcacagggaaaaggctatccggacctcaatacgaggaacctggtgtattgtcttcgagacgcgcgtccgtggatcccgatttacaccttggtcgattatgaccctgacgggatcagaatactgtgcacgtataaatacggcagctcttctttggagcacgagagacgatcggctgtgaacagcatcgagtggataggaattcgcttttcggacgtcaaacagcactatctgagaccatgcaacagtctcttgcaggatgatggctcccaaatcaacattgaaggtacgtgccatcacaaagaaagtcaccctcaacaaggaagactttccaagccaagaagctgcggccctccataccaagggctgcgacgctgagaccaggagcctctatctaactcaagtactctccaatatgtagcacactcaagattggacgtagtacaggtcagaagtcggccaggattttctatgccacgacagaacgatttcgaagcaagcacgtcccagctgacaaccagggaccgtaaacttgcccatgagatggtttcaaggctatctggatcattagatatgaggggagaacatgaagagcacttgcgcgagcttcaggtcatgcttatgctcaatgtcaaggccgagatacaagctgttgacaatcttggggatattaccgagtggattgacaacaaactttgcgcccagctgatgggtgcatag